European Patent Specification EP 3 328 427 B1, published May 29, 2024. Title: ANTIBODY DERIVATIVES WITH CONDITIONALLY ENABLED EFFECTOR FUNCTION. Applicant: THE GENERAL HOSPITAL CORPORATION. The sequence listing filed with the application follows.

SEQUENCE LISTING (71 sequences)

SEQ ID NO: 1 - DNA, 1530 bp, Artificial Sequence
  Description of Artificial Sequence: Synthetic polynucleotide
ggtaccgccgccaccatggactggacctggaggattctcttcttggtggcagcagccacaggagcccactcccaggtgcagctgcagcagcccggcgccgagttagttaaacccggcgccagcgtgaagatgagctgcaaggccagcggctacaccttcaccagctacaacatgcactgggtgaagcagacccccggcaggggcctggagtggatcggcgccatctaccccggcaacggcgacaccagctacaaccagaagttcaagggcaaggccaccctgaccgccgacaagagcagcagcaccgcctacatgcagctgagcagcctgaccagcgaggacagcgccgtgtactactgcgccaggagcacctactacggcggcgactggtacttcaacgtgtggggcgccggcaccaccgtgaccgtgagcgccgcctccaccaagggcccatcggtcttccccctggcaccctcctccaagagcacctctgggggcacagcggccctgggctgcctggtcaaggactacttccccgagccggtgacggtgtcgtggaactcaggcgccctgaccagcggcgtgcacaccttcccggctgtcctacagtcctcaggactctactccctctcttccgtggtgaccgtgccctccagcagcttgggcacccagacctacatctgcaacgtgaatcacaagcccagcaacaccaaggtggacaagaaagttgagcccaaatcttgtgacaaaactcacacatgcccaccgtgcccagcacctgaactcctggggggaccgtcagtcttcctcttccccccaaaacccaaggacaccctcatgatctcccggacccctgaggtcacatgcgtggtggtggacgtgagccacgaagaccctgaggtcaagttcaactggtacgtggacggcgtggaggtgcataatgccaagacaaagccgcgggaggagcagtacaacagcacgtaccgggtggtcagcgtcctcaccgtcctgcaccaggactggctgaatggcaaggagtacaagtgcaaagtctccaacaaagccctgcctgcccccatcgagaaaaccatctccaaagccaaagggcagccccgagaaccacaggtgtacaccctgcccccatcccgggatgagctgaccaagaaccaggtcagcctgacctgcctggtcaaaggcttctatcccagcgacatcgccgtggagtgggagagcaatgggcagccggagaacaactacaagaccacgcctcccgtgctggactccgacggctccttcttcctctactcaaagctcaccgtggacaagagcaggtggcagcaggggaacgtcttctcatgctccgtgatgcatgaggctctgcacaaccactacacgcagaagagcctctccctgtctccgggtaaaggtggaggtggttcacatcatcaccatcatcaccctggcggaggactaaacgacatcttcgaggctcagaaaatcgaatggcacgaaggtccttgataatctaga

SEQ ID NO: 2 - protein, 501 aa, Artificial Sequence
  Description of Artificial Sequence: Synthetic polypeptide
MDWTWRILFLVAAATGAHSQVQLQQPGAELVKPGASVKMSCKASGYTFTSYNMHWVKQTPGRGLEWIGAIYPGNGDTSYNQKFKGKATLTADKSSSTAYMQLSSLTSEDSAVYYCARSTYYGGDWYFNVWGAGTTVTVSAASTKGPSVFPLAPSSKSTSGGTAALGCLVKDYFPEPVTVSWNSGALTSGVHTFPAVLQSSGLYSLSSVVTVPSSSLGTQTYICNVNHKPSNTKVDKKVEPKSCDKTHTCPPCPAPELLGGPSVFLFPPKPKDTLMISRTPEVTCVVVDVSHEDPEVKFNWYVDGVEVHNAKTKPREEQYNSTYRVVSVLTVLHQDWLNGKEYKCKVSNKALPAPIEKTISKAKGQPREPQVYTLPPSRDELTKNQVSLTCLVKGFYPSDIAVEWESNGQPENNYKTTPPVLDSDGSFFLYSKLTVDKSRWQQGNVFSCSVMHEALHNHYTQKSLSLSPGKGGGGSHHHHHHPGGGLNDIFEAQKIEWHEGP

SEQ ID NO: 3 - DNA, 723 bp, Artificial Sequence
  Description of Artificial Sequence: Synthetic polynucleotide
ggtaccgccgccaccatggactggacctggaggattctcttcttggtggcagcagccacaggagcccactcccagatcgtgctgagccagagccccgccatcctgagcgccagccccggcgagaaggtgaccatgacctgcagggccagcagcagcgtgagctacatccactggttccagcagaagcccggcagcagccccaagccctggatctacgccaccagcaacctggccagcggcgtgcccgtgaggttcagcggcagcggcagcggcaccagctacagcctgaccatcagcagggtggaggccgaggacgccgccacctactactgccagcagtggaccagcaacccccccaccttcggcggcggcaccaagctggagatcaagaggaccgtggccgcccccagcgtgttcatcttcccaccatctgacgagcagctgaagagcggcaccgccagcgtggtgtgcctgctgaacaacttctaccccagggaggccaaggtgcagtggaaggtggacaacgccctgcagagcggcaacagccaggagagcgtgaccgagcaggacagcaaggacagcacctacagcctgagcagcaccctgaccctgagcaaggccgactacgagaagcacaaggtgtacgcctgcgaggtgacccaccagggcctgagcagccccgtgaccaagagcttcaacaggggcgagtgctgataatctaga

SEQ ID NO: 4 - protein, 232 aa, Artificial Sequence
  Description of Artificial Sequence: Synthetic polypeptide
MDWTWRILFLVAAATGAHSQIVLSQSPAILSASPGEKVTMTCRASSSVSYIHWFQQKPGSSPKPWIYATSNLASGVPVRFSGSGSGTSYSLTISRVEAEDAATYYCQQWTSNPPTFGGGTKLEIKRTVAAPSVFIFPPSDEQLKSGTASVVCLLNNFYPREAKVQWKVDNALQSGNSQESVTEQDSKDSTYSLSSTLTLSKADYEKHKVYACEVTHQGLSSPVTKSFNRGEC

SEQ ID NO: 5 - DNA, 2283 bp, Artificial Sequence
  Description of Artificial Sequence: Synthetic polynucleotide
ggtaccgccgccaccatggactggacctggaggattctcttcttggtggcagcagccacaggagcccactcccaggtgcagctgcagcagcccggcgccgagttagttaaacccggcgccagcgtgaagatgagctgcaaggccagcggctacaccttcaccagctacaacatgcactgggtgaagcagacccccggcaggggcctggagtggatcggcgccatctaccccggcaacggcgacaccagctacaaccagaagttcaagggcaaggccaccctgaccgccgacaagagcagcagcaccgcctacatgcagctgagcagcctgaccagcgaggacagcgccgtgtactactgcgccaggagcacctactacggcggcgactggtacttcaacgtgtggggcgccggcaccaccgtgaccgtgagcgccgcctccaccaagggcccatcggtcttccccctggcaccctcctccaagagcacctctgggggcacagcggccctgggctgcctggtcaaggactacttccccgagccggtgacggtgtcgtggaactcaggcgccctgaccagcggcgtgcacaccttcccggctgtcctacagtcctcaggactctactccctctcttccgtggtgaccgtgccctccagcagcttgggcacccagacctacatctgcaacgtgaatcacaagcccagcaacaccaaggtggacaagaaagttgagcccaaatcttgtgacaaaactcacacatgcccaccgtgcccagcacctgaactcctggggggaccgtcagtcttcctcttccccccaaaacccaaggacaccctcatgatctcccggacccctgaggtcacatgcgtggtggtggacgtgagccacgaagaccctgaggtcaagttcaactggtacgtggacggcgtggaggtgcataatgccaagacaaagccgcgggaggagcagtacaacagcacgtaccgggtggtcagcgtcctcaccgtcctgcaccaggactggctgaatggcaaggagtacaagtgcaaagtctccaacaaagccctgcctgcccccatcgagaaaaccatctccaaagccaaagggcagccccgagaaccacaggtgtacaccctgcccccatcccgggatgagctgaccaagaaccaggtcagcctgacctgcctggtcaaaggcttctatcccagcgacatcgccgtggagtgggagagcaatgggcagccggagaacaactacaagaccacgcctcccgtgctggactccgacggctccttcttcctctactcaaagctcaccgtggacaagagcaggtggcagcaggggaacgtcttctcatgctccgtgatgcatgaggctctgcacaaccactacacgcagaagagcctctccctgtctccgggtaaaggtggaggtggttcacatcatcaccatcatcaccctggcggaggactaaacgacatcttcgaggctcagaaaatcgaatggcacgaaggtcctgaattcggcggaggcggctccggcggaggcggcgaatccggcggaggcggctccggaggcggcggctccgaaggcggcggaggtattgaaccttttagcggtggaggtggctccgaaggcggtggcggctccggaggcggcggcgaatccggcggcggcggatctggaggcggcggcgaatccggcgcgcccggtagcactagtggtattataccttttagcgcggccgcacctggcggaggcccaaaggctgtggtgttcctggagcctcaatggtacagcgtgcttgagaaggacagtgtgactctgaagtgccagggagcctactcccctgaggacaattccacacagtggtttcacaatgagagcctcatctcaagccaggcctcgagctacttcattgacgctgccacagtcaacgacagtggagagtacaggtgccagacaaacctctccaccctcagtgacccggtgcagctagaagtccatatcggctggctgttgctccaggcccctcggtgggtgttcaaggaggaagaccctattcacctgaggtgtcacagctggaagaacactgctctgcataaggtcacatatttacagaatggcaaagacaggaagtattttcatcataattctgacttccacattccaaaagccacactcaaagatagcggctcctacttctgcagggggcttgttgggagtaaaaatgtgtcttcagagactgtgaacatcaccatcactcaaggttgataatctaga

SEQ ID NO: 6 - protein, 752 aa, Artificial Sequence
  Description of Artificial Sequence: Synthetic polypeptide
MDWTWRILFLVAAATGAHSQVQLQQPGAELVKPGASVKMSCKASGYTFTSYNMHWVKQTPGRGLEWIGAIYPGNGDTSYNQKFKGKATLTADKSSSTAYMQLSSLTSEDSAVYYCARSTYYGGDWYFNVWGAGTTVTVSAASTKGPSVFPLAPSSKSTSGGTAALGCLVKDYFPEPVTVSWNSGALTSGVHTFPAVLQSSGLYSLSSVVTVPSSSLGTQTYICNVNHKPSNTKVDKKVEPKSCDKTHTCPPCPAPELLGGPSVFLFPPKPKDTLMISRTPEVTCVVVDVSHEDPEVKFNWYVDGVEVHNAKTKPREEQYNSTYRVVSVLTVLHQDWLNGKEYKCKVSNKALPAPIEKTISKAKGQPREPQVYTLPPSRDELTKNQVSLTCLVKGFYPSDIAVEWESNGQPENNYKTTPPVLDSDGSFFLYSKLTVDKSRWQQGNVFSCSVMHEALHNHYTQKSLSLSPGKGGGGSHHHHHHPGGGLNDIFEAQKIEWHEGPEFGGGGSGGGGESGGGGSGGGGSEGGGGIEPFSGGGGSEGGGGSGGGGESGGGGSGGGGESGAPGSTSGIIPFSAAAPGGGPKAVVFLEPQWYSVLEKDSVTLKCQGAYSPEDNSTQWFHNESLISSQASSYFIDAATVNDSGEYRCQTNLSTLSDPVQLEVHIGWLLLQAPRWVFKEEDPIHLRCHSWKNTALHKVTYLQNGKDRKYFHHNSDFHIPKATLKDSGSYFCRGLVGSKNVSSETVNITITQG

SEQ ID NO: 7 - DNA, 2283 bp, Artificial Sequence
  Description of Artificial Sequence: Synthetic polynucleotide
ggtaccgccgccaccatggactggacctggaggattctcttcttggtggcagcagccacaggagcccactcccaggtgcagctgcagcagcccggcgccgagttagttaaacccggcgccagcgtgaagatgagctgcaaggccagcggctacaccttcaccagctacaacatgcactgggtgaagcagacccccggcaggggcctggagtggatcggcgccatctaccccggcaacggcgacaccagctacaaccagaagttcaagggcaaggccaccctgaccgccgacaagagcagcagcaccgcctacatgcagctgagcagcctgaccagcgaggacagcgccgtgtactactgcgccaggagcacctactacggcggcgactggtacttcaacgtgtggggcgccggcaccaccgtgaccgtgagcgccgcctccaccaagggcccatcggtcttccccctggcaccctcctccaagagcacctctgggggcacagcggccctgggctgcctggtcaaggactacttccccgagccggtgacggtgtcgtggaactcaggcgccctgaccagcggcgtgcacaccttcccggctgtcctacagtcctcaggactctactccctctcttccgtggtgaccgtgccctccagcagcttgggcacccagacctacatctgcaacgtgaatcacaagcccagcaacaccaaggtggacaagaaagttgagcccaaatcttgtgacaaaactcacacatgcccaccgtgcccagcacctgaactcctggggggaccgtcagtcttcctcttccccccaaaacccaaggacaccctcatgatctcccggacccctgaggtcacatgcgtggtggtggacgtgagccacgaagaccctgaggtcaagttcaactggtacgtggacggcgtggaggtgcataatgccaagacaaagccgcgggaggagcagtacaacagcacgtaccgggtggtcagcgtcctcaccgtcctgcaccaggactggctgaatggcaaggagtacaagtgcaaagtctccaacaaagccctgcctgcccccatcgagaaaaccatctccaaagccaaagggcagccccgagaaccacaggtgtacaccctgcccccatcccgggatgagctgaccaagaaccaggtcagcctgacctgcctggtcaaaggcttctatcccagcgacatcgccgtggagtgggagagcaatgggcagccggagaacaactacaagaccacgcctcccgtgctggactccgacggctccttcttcctctactcaaagctcaccgtggacaagagcaggtggcagcaggggaacgtcttctcatgctccgtgatgcatgaggctctgcacaaccactacacgcagaagagcctctccctgtctccgggtaaaggtggaggtggttcacatcatcaccatcatcaccctggcggaggactaaacgacatcttcgaggctcagaaaatcgaatggcacgaaggtcctgaattcggcggaggcggctccggcggaggcggcgaatccggcggaggcggctccggaggcggcggctccgaaggcggcggaggtattgaaccttttagcggtggaggtggctccgaaggcggtggcggctccggaggcggcggcgaatccggcggcggcggatctggaggcggcggcgaatccggcgcgcccggtagcactagtggtattataccttttagcgcggccgcacctggcggaggcccaaaggctgtgctgaaacttgagcccccgtggatcaacgtgctccaggaggactctgtgactctgacatgccagggggctcgcagccctgagagcgactccattcagtggttccacaatgggaatctcattcccacccacacgcagcccagctacaggttcaaggccaacaacaatgacagcggggagtacacgtgccagactggccagaccagcctcagcgaccctgtgcatctgactgtgctttccgaatggctggtgctccagacccctcacctggagttccaggagggagaaaccatcatgctgaggtgccacagctggaaggacaagcctctggtcaaggtcacattcttccagaatggaaaatcccagaaattctcccgtttggatcccaccttctccatcccacaagcaaaccacagtcacagtggtgattaccactgcacaggaaacataggctacacgctgttctcatccaagcctgtgaccatcactgtccaagtgccctgataatctaga

SEQ ID NO: 8 - protein, 752 aa, Artificial Sequence
  Description of Artificial Sequence: Synthetic polypeptide
MDWTWRILFLVAAATGAHSQVQLQQPGAELVKPGASVKMSCKASGYTFTSYNMHWVKQTPGRGLEWIGAIYPGNGDTSYNQKFKGKATLTADKSSSTAYMQLSSLTSEDSAVYYCARSTYYGGDWYFNVWGAGTTVTVSAASTKGPSVFPLAPSSKSTSGGTAALGCLVKDYFPEPVTVSWNSGALTSGVHTFPAVLQSSGLYSLSSVVTVPSSSLGTQTYICNVNHKPSNTKVDKKVEPKSCDKTHTCPPCPAPELLGGPSVFLFPPKPKDTLMISRTPEVTCVVVDVSHEDPEVKFNWYVDGVEVHNAKTKPREEQYNSTYRVVSVLTVLHQDWLNGKEYKCKVSNKALPAPIEKTISKAKGQPREPQVYTLPPSRDELTKNQVSLTCLVKGFYPSDIAVEWESNGQPENNYKTTPPVLDSDGSFFLYSKLTVDKSRWQQGNVFSCSVMHEALHNHYTQKSLSLSPGKGGGGSHHHHHHPGGGLNDIFEAQKIEWHEGPEFGGGGSGGGGESGGGGSGGGGSEGGGGIEPFSGGGGSEGGGGSGGGGESGGGGSGGGGESGAPGSTSGIIPFSAAAPGGGPKAVLKLEPPWINVLQEDSVTLTCQGARSPESDSIQWFHNGNLIPTHTQPSYRFKANNNDSGEYTCQTGQTSLSDPVHLTVLSEWLVLQTPHLEFQEGETIMLRCHSWKDKPLVKVTFFQNGKSQKFSRLDPTFSIPQANHSHSGDYHCTGNIGYTLFSSKPVTITVQVP

SEQ ID NO: 9 - DNA, 2286 bp, Artificial Sequence
  Description of Artificial Sequence: Synthetic polynucleotide
ggtaccgccgccaccatggactggacctggaggattctcttcttggtggcagcagccacaggagcccactcccaggtgcagctgcagcagcccggcgccgagttagttaaacccggcgccagcgtgaagatgagctgcaaggccagcggctacaccttcaccagctacaacatgcactgggtgaagcagacccccggcaggggcctggagtggatcggcgccatctaccccggcaacggcgacaccagctacaaccagaagttcaagggcaaggccaccctgaccgccgacaagagcagcagcaccgcctacatgcagctgagcagcctgaccagcgaggacagcgccgtgtactactgcgccaggagcacctactacggcggcgactggtacttcaacgtgtggggcgccggcaccaccgtgaccgtgagcgccgcctccaccaagggcccatcggtcttccccctggcaccctcctccaagagcacctctgggggcacagcggccctgggctgcctggtcaaggactacttccccgagccggtgacggtgtcgtggaactcaggcgccctgaccagcggcgtgcacaccttcccggctgtcctacagtcctcaggactctactccctctcttccgtggtgaccgtgccctccagcagcttgggcacccagacctacatctgcaacgtgaatcacaagcccagcaacaccaaggtggacaagaaagttgagcccaaatcttgtgacaaaactcacacatgcccaccgtgcccagcacctgaactcctggggggaccgtcagtcttcctcttccccccaaaacccaaggacaccctcatgatctcccggacccctgaggtcacatgcgtggtggtggacgtgagccacgaagaccctgaggtcaagttcaactggtacgtggacggcgtggaggtgcataatgccaagacaaagccgcgggaggagcagtacaacagcacgtaccgggtggtcagcgtcctcaccgtcctgcaccaggactggctgaatggcaaggagtacaagtgcaaagtctccaacaaagccctgcctgcccccatcgagaaaaccatctccaaagccaaagggcagccccgagaaccacaggtgtacaccctgcccccatcccgggatgagctgaccaagaaccaggtcagcctgacctgcctggtcaaaggcttctatcccagcgacatcgccgtggagtgggagagcaatgggcagccggagaacaactacaagaccacgcctcccgtgctggactccgacggctccttcttcctctactcaaagctcaccgtggacaagagcaggtggcagcaggggaacgtcttctcatgctccgtgatgcatgaggctctgcacaaccactacacgcagaagagcctctccctgtctccgggtaaaggtggaggtggttcacatcatcaccatcatcaccctggcggaggactaaacgacatcttcgaggctcagaaaatcgaatggcacgaaggtcctgaattcggcggaggcggctccggcggaggcggcgaatccggcggaggcggctccggaggcggcggctccgaaggcggcggaggtattgaaccttttagcggtggaggtggctccgaaggcggtggcggctccggaggcggcggcgaatccggcggcggcggatctggaggcggcggcgaatccggcgcgcccggtagcactagtggtattataccttttagcgcggccgcacctggcggaggcacaaaggcagtgatcactttgcagcctccatgggtcagcgtgttccaagaggaaaccgtaaccttgcactgtgaggtgctccatctgcctgggagcagctctacacagtggtttctcaatggcacagccactcagacctcgacccccagctacagaatcacctctgccagtgtcaatgacagtggtgaatacaggtgccagagaggtctctcagggcgaagtgaccccatacagctggaaatccacagaggctggctactactgcaggtctccagcagagtcttcacggaaggagaacctctggccttgaggtgtcatgcgtggaaggataagctggtgtacaatgtgctttactatcgaaatggcaaagcctttaagtttttccactggaattctaacctcaccattctgaaaaccaacataagtcacaatggcacctaccattgctcaggcatgggaaagcatcgctacacatcagcaggaatatctgtcactgtgaaagagctatttccatgataatctaga

SEQ ID NO: 10 - protein, 753 aa, Artificial Sequence
  Description of Artificial Sequence: Synthetic polypeptide
MDWTWRILFLVAAATGAHSQVQLQQPGAELVKPGASVKMSCKASGYTFTSYNMHWVKQTPGRGLEWIGAIYPGNGDTSYNQKFKGKATLTADKSSSTAYMQLSSLTSEDSAVYYCARSTYYGGDWYFNVWGAGTTVTVSAASTKGPSVFPLAPSSKSTSGGTAALGCLVKDYFPEPVTVSWNSGALTSGVHTFPAVLQSSGLYSLSSVVTVPSSSLGTQTYICNVNHKPSNTKVDKKVEPKSCDKTHTCPPCPAPELLGGPSVFLFPPKPKDTLMISRTPEVTCVVVDVSHEDPEVKFNWYVDGVEVHNAKTKPREEQYNSTYRVVSVLTVLHQDWLNGKEYKCKVSNKALPAPIEKTISKAKGQPREPQVYTLPPSRDELTKNQVSLTCLVKGFYPSDIAVEWESNGQPENNYKTTPPVLDSDGSFFLYSKLTVDKSRWQQGNVFSCSVMHEALHNHYTQKSLSLSPGKGGGGSHHHHHHPGGGLNDIFEAQKIEWHEGPEFGGGGSGGGGESGGGGSGGGGSEGGGGIEPFSGGGGSEGGGGSGGGGESGGGGSGGGGESGAPGSTSGIIPFSAAAPGGGTKAVITLQPPWVSVFQEETVTLHCEVLHLPGSSSTQWFLNGTATQTSTPSYRITSASVNDSGEYRCQRGLSGRSDPIQLEIHRGWLLLQVSSRVFTEGEPLALRCHAWKDKLVYNVLYYRNGKAFKFFHWNSNLTILKTNISHNGTYHCSGMGKHRYTSAGISVTVKELFP

SEQ ID NO: 11 - DNA, 1386 bp, Artificial Sequence
  Description of Artificial Sequence: Synthetic polynucleotide
ggtaccgccgccaccatggactggacctggaggattctcttcttggtggcagcagccacaggagcccactcccagatcgtgctgagccagagccccgccatcctgagcgccagccccggcgagaaggtgaccatgacctgcagggccagcagcagcgtgagctacatccactggttccagcagaagcccggcagcagccccaagccctggatctacgccaccagcaacctggccagcggcgtgcccgtgaggttcagcggcagcggcagcggcaccagctacagcctgaccatcagcagggtggaggccgaggacgccgccacctactactgccagcagtggaccagcaacccccccaccttcggcggcggcaccaagctggagatcaagaggaccgtggccgcccccagcgtgttcatcttcccaccatctgacgagcagctgaagagcggcaccgccagcgtggtgtgcctgctgaacaacttctaccccagggaggccaaggtgcagtggaaggtggacaacgccctgcagagcggcaacagccaggagagcgtgaccgagcaggacagcaaggacagcacctacagcctgagcagcaccctgaccctgagcaaggccgactacgagaagcacaaggtgtacgcctgcgaggtgacccaccagggcctgagcagccccgtgaccaagagcttcaacaggggcgagtgcggtggaggtggatcagaattctccccaggcggcggctccgaaggcggcggaggtattgaaccttttagcggtggaggtggctccgaaggcggtggcgcgcccggtagcactagtggtattataccttttagcgcggccgcacctggcggaggcccaaaggctgtggtgttcctggagcctcaatggtacagcgtgcttgagaaggacagtgtgactctgaagtgccagggagcctactcccctgaggacaattccacacagtggtttcacaatgagagcctcatctcaagccaggcctcgagctacttcattgacgctgccacagtcaacgacagtggagagtacaggtgccagacaaacctctccaccctcagtgacccggtgcagctagaagtccatatcggctggctgttgctccaggcccctcggtgggtgttcaaggaggaagaccctattcacctgaggtgtcacagctggaagaacactgctctgcataaggtcacatatttacagaatggcaaagacaggaagtattttcatcataattctgacttccacattccaaaagccacactcaaagatagcggctcctacttctgcagggggcttgttgggagtaaaaatgtgtcttcagagactgtgaacatcaccatcactcaaggttgataatctaga

SEQ ID NO: 12 - protein, 453 aa, Artificial Sequence
  Description of Artificial Sequence: Synthetic polypeptide
MDWTWRILFLVAAATGAHSQIVLSQSPAILSASPGEKVTMTCRASSSVSYIHWFQQKPGSSPKPWIYATSNLASGVPVRFSGSGSGTSYSLTISRVEAEDAATYYCQQWTSNPPTFGGGTKLEIKRTVAAPSVFIFPPSDEQLKSGTASVVCLLNNFYPREAKVQWKVDNALQSGNSQESVTEQDSKDSTYSLSSTLTLSKADYEKHKVYACEVTHQGLSSPVTKSFNRGECGGGGSEFSPGGGSEGGGGIEPFSGGGGSEGGGAPGSTSGIIPFSAAAPGGGPKAVVFLEPQWYSVLEKDSVTLKCQGAYSPEDNSTQWFHNESLISSQASSYFIDAATVNDSGEYRCQTNLSTLSDPVQLEVHIGWLLLQAPRWVFKEEDPIHLRCHSWKNTALHKVTYLQNGKDRKYFHHNSDFHIPKATLKDSGSYFCRGLVGSKNVSSETVNITITQG

SEQ ID NO: 13 - DNA, 1386 bp, Artificial Sequence
  Description of Artificial Sequence: Synthetic polynucleotide
ggtaccgccgccaccatggactggacctggaggattctcttcttggtggcagcagccacaggagcccactcccagatcgtgctgagccagagccccgccatcctgagcgccagccccggcgagaaggtgaccatgacctgcagggccagcagcagcgtgagctacatccactggttccagcagaagcccggcagcagccccaagccctggatctacgccaccagcaacctggccagcggcgtgcccgtgaggttcagcggcagcggcagcggcaccagctacagcctgaccatcagcagggtggaggccgaggacgccgccacctactactgccagcagtggaccagcaacccccccaccttcggcggcggcaccaagctggagatcaagaggaccgtggccgcccccagcgtgttcatcttcccaccatctgacgagcagctgaagagcggcaccgccagcgtggtgtgcctgctgaacaacttctaccccagggaggccaaggtgcagtggaaggtggacaacgccctgcagagcggcaacagccaggagagcgtgaccgagcaggacagcaaggacagcacctacagcctgagcagcaccctgaccctgagcaaggccgactacgagaagcacaaggtgtacgcctgcgaggtgacccaccagggcctgagcagccccgtgaccaagagcttcaacaggggcgagtgcggtggaggtggatcagaattctccccaggcggcggctccgaaggcggcggaggtattgaaccttttagcggtggaggtggctccgaaggcggtggcgcgcccggtagcactagtggtattataccttttagcgcggccgcacctggcggaggcccaaaggctgtgctgaaacttgagcccccgtggatcaacgtgctccaggaggactctgtgactctgacatgccagggggctcgcagccctgagagcgactccattcagtggttccacaatgggaatctcattcccacccacacgcagcccagctacaggttcaaggccaacaacaatgacagcggggagtacacgtgccagactggccagaccagcctcagcgaccctgtgcatctgactgtgctttccgaatggctggtgctccagacccctcacctggagttccaggagggagaaaccatcatgctgaggtgccacagctggaaggacaagcctctggtcaaggtcacattcttccagaatggaaaatcccagaaattctcccgtttggatcccaccttctccatcccacaagcaaaccacagtcacagtggtgattaccactgcacaggaaacataggctacacgctgttctcatccaagcctgtgaccatcactgtccaagtgccctgataatctaga

SEQ ID NO: 14 - protein, 453 aa, Artificial Sequence
  Description of Artificial Sequence: Synthetic polypeptide
MDWTWRILFLVAAATGAHSQIVLSQSPAILSASPGEKVTMTCRASSSVSYIHWFQQKPGSSPKPWIYATSNLASGVPVRFSGSGSGTSYSLTISRVEAEDAATYYCQQWTSNPPTFGGGTKLEIKRTVAAPSVFIFPPSDEQLKSGTASVVCLLNNFYPREAKVQWKVDNALQSGNSQESVTEQDSKDSTYSLSSTLTLSKADYEKHKVYACEVTHQGLSSPVTKSFNRGECGGGGSEFSPGGGSEGGGGIEPFSGGGGSEGGGAPGSTSGIIPFSAAAPGGGPKAVLKLEPPWINVLQEDSVTLTCQGARSPESDSIQWFHNGNLIPTHTQPSYRFKANNNDSGEYTCQTGQTSLSDPVHLTVLSEWLVLQTPHLEFQEGETIMLRCHSWKDKPLVKVTFFQNGKSQKFSRLDPTFSIPQANHSHSGDYHCTGNIGYTLFSSKPVTITVQVP

SEQ ID NO: 15 - DNA, 1389 bp, Artificial Sequence
  Description of Artificial Sequence: Synthetic polynucleotide
ggtaccgccgccaccatggactggacctggaggattctcttcttggtggcagcagccacaggagcccactcccagatcgtgctgagccagagccccgccatcctgagcgccagccccggcgagaaggtgaccatgacctgcagggccagcagcagcgtgagctacatccactggttccagcagaagcccggcagcagccccaagccctggatctacgccaccagcaacctggccagcggcgtgcccgtgaggttcagcggcagcggcagcggcaccagctacagcctgaccatcagcagggtggaggccgaggacgccgccacctactactgccagcagtggaccagcaacccccccaccttcggcggcggcaccaagctggagatcaagaggaccgtggccgcccccagcgtgttcatcttcccaccatctgacgagcagctgaagagcggcaccgccagcgtggtgtgcctgctgaacaacttctaccccagggaggccaaggtgcagtggaaggtggacaacgccctgcagagcggcaacagccaggagagcgtgaccgagcaggacagcaaggacagcacctacagcctgagcagcaccctgaccctgagcaaggccgactacgagaagcacaaggtgtacgcctgcgaggtgacccaccagggcctgagcagccccgtgaccaagagcttcaacaggggcgagtgcggtggaggtggatcagaattctccccaggcggcggctccgaaggcggcggaggtattgaaccttttagcggtggaggtggctccgaaggcggtggcgcgcccggtagcactagtggtattataccttttagcgcggccgcacctggcggaggcacaaaggcagtgatcactttgcagcctccatgggtcagcgtgttccaagaggaaaccgtaaccttgcactgtgaggtgctccatctgcctgggagcagctctacacagtggtttctcaatggcacagccactcagacctcgacccccagctacagaatcacctctgccagtgtcaatgacagtggtgaatacaggtgccagagaggtctctcagggcgaagtgaccccatacagctggaaatccacagaggctggctactactgcaggtctccagcagagtcttcacggaaggagaacctctggccttgaggtgtcatgcgtggaaggataagctggtgtacaatgtgctttactatcgaaatggcaaagcctttaagtttttccactggaattctaacctcaccattctgaaaaccaacataagtcacaatggcacctaccattgctcaggcatgggaaagcatcgctacacatcagcaggaatatctgtcactgtgaaagagctatttccatgataatctaga

SEQ ID NO: 16 - protein, 454 aa, Artificial Sequence
  Description of Artificial Sequence: Synthetic polypeptide
MDWTWRILFLVAAATGAHSQIVLSQSPAILSASPGEKVTMTCRASSSVSYIHWFQQKPGSSPKPWIYATSNLASGVPVRFSGSGSGTSYSLTISRVEAEDAATYYCQQWTSNPPTFGGGTKLEIKRTVAAPSVFIFPPSDEQLKSGTASVVCLLNNFYPREAKVQWKVDNALQSGNSQESVTEQDSKDSTYSLSSTLTLSKADYEKHKVYACEVTHQGLSSPVTKSFNRGECGGGGSEFSPGGGSEGGGGIEPFSGGGGSEGGGAPGSTSGIIPFSAAAPGGGTKAVITLQPPWVSVFQEETVTLHCEVLHLPGSSSTQWFLNGTATQTSTPSYRITSASVNDSGEYRCQRGLSGRSDPIQLEIHRGWLLLQVSSRVFTEGEPLALRCHAWKDKLVYNVLYYRNGKAFKFFHWNSNLTILKTNISHNGTYHCSGMGKHRYTSAGISVTVKELFP

SEQ ID NO: 17 - DNA, 777 bp, Artificial Sequence
  Description of Artificial Sequence: Synthetic polynucleotide
ccatggataatataaatcgcgctcgcaaaaagcgcgttatcggtggtcatgaagctaaaccgcactcccgtccgtacatggcttacctgatgatctctggtccaagcggttcgaaacgttgcggtggtttcctgatccaggacgacttcgttctgaccgctgctcactgctggggttcctccatcaacgttaccctgggtgctcacaacatcaaagaacaggaaccgacccagcagttcatcccggttaaacgtgctatcccgcacccggcttacaacccgaaaaacttctccaacgacatcatgctgctgcagctggaacagaaagctaaacagacccaggctgttcagccgctgcgtctgccgtccaacaaagctcaggttaaaccgggtcagacctgctccgttgctggttggggtcagaccgctccgctgggtaaacactcccacactctgcaggaagttaaaatgaccgttcaggaagatcgtaaatgcgaatccgacctgcgtcactactacgactccaccatcgaactgtgcgttggtgatccggaaatcaaaaaaacctccttcaaaggtgactccggtggtccgctggtttgcaacaaagttgctcagggtatcgtttcctacggtcgtaccaacggtatgccgccgatcgcttacaccaaagtttcctccttcgttcactggatcgaaaaaactatggaacgttacaccggttccggactgcctgagactggaagcggccaccaccatcatcaccattagcggccgc

SEQ ID NO: 18 - protein, 255 aa, Artificial Sequence
  Description of Artificial Sequence: Synthetic polypeptide
MDNINRARKKRVIGGHEAKPHSRPYMAYLMISGPSGSKRCGGFLIQDDFVLTAAHCWGSSINVTLGAHNIKEQEPTQQFIPVKRAIPHPAYNPKNFSNDIMLLQLEQKAKQTQAVQPLRLPSNKAQVKPGQTCSVAGWGQTAPLGKHSHTLQEVKMTVQEDRKCESDLRHYYDSTIELCVGDPEIKKTSFKGDSGGPLVCNKVAQGIVSYGRTNGMPPIAYTKVSSFVHWIEKTMERYTGSGLPETGSGHHHHHH

SEQ ID NO: 19 - DNA, 900 bp, Artificial Sequence
  Description of Artificial Sequence: Synthetic polynucleotide
atgaaatacctgctgccgaccgctgctgctggtctgctgctcctcgctgcccagccggcgatggccggtaaaggtggtggctctccagctagccaggtgcagctgcagcagtccggcccgggcatcgtgaaaccgagccagaccctgaccctgacctgctccttcagcggcttctccctgtccaccccgggcatgggcgtttcctggattcgccagccgccgggcaaagcgccagagtggctggctcacatctactgggacgacgacaaacgctacaacccgcagctgaaatcccgcctgactatctccaaagacacctccaaaaaccaggttgtgctgaccatgaccaacatggacagcgaggacaccgctacctactactgcacccgccgcgttccgtcccgggttatgaccacctccggctacttcgacgtttggggccagggcaccacggtgaccgtgagcagcggtggcggcggtagcggtggtggcggcagcggcggtggcggtagcgggagctccgacatcgttctgacccagtccccggattccctggctgtttccctgggcgaacgcgctaccatcaactgccgcgcttcccagtccgtttccacctccacctactcctacatgcactggtaccagcagaaaccgggccagccgccgaaactgctgatcaaatacgcttccaacctggagtccggcgttccggctcgcttctccggctccggctccgaaaccgacttcaccctgaccatccacagcatggagccggaagacttcgctacctactactgccagcactcctgggagaacccgtggaccttcggcggcggcaccaaagtggagatcaagggggatccggcggccgcactcgagcaccaccaccaccaccactga

SEQ ID NO: 20 - protein, 299 aa, Artificial Sequence
  Description of Artificial Sequence: Synthetic polypeptide
MKYLLPTAAAGLLLLAAQPAMAGKGGGSPASQVQLQQSGPGIVKPSQTLTLTCSFSGFSLSTPGMGVSWIRQPPGKAPEWLAHIYWDDDKRYNPQLKSRLTISKDTSKNQVVLTMTNMDSEDTATYYCTRRVPSRVMTTSGYFDVWGQGTTVTVSSGGGGSGGGGSGGGGSGSSDIVLTQSPDSLAVSLGERATINCRASQSVSTSTYSYMHWYQQKPGQPPKLLIKYASNLESGVPARFSGSGSETDFTLTIHSMEPEDFATYYCQHSWENPWTFGGGTKVEIKGDPAAALEHHHHHH

SEQ ID NO: 21 - protein, 523 aa, Artificial Sequence
  Description of Artificial Sequence: Synthetic polypeptide
MDNINRARKKRVIGGHEAKPHSRPYMAYLMISGPSGSKRCGGFLIQDDFVLTAAHCWGSSINVTLGAHNIKEQEPTQQFIPVKRAIPHPAYNPKNFSNDIMLLQLEQKAKQTQAVQPLRLPSNKAQVKPGQTCSVAGWGQTAPLGKHSHTLQEVKMTVQEDRKCESDLRHYYDSTIELCVGDPEIKKTSFKGDSGGPLVCNKVAQGIVSYGRTNGMPPIAYTKVSSFVHWIEKTMERYTGSGLPETGKGGGSPASQVQLQQSGPGIVKPSQTLTLTCSFSGFSLSTPGMGVSWIRQPPGKAPEWLAHIYWDDDKRYNPQLKSRLTISKDTSKNQVVLTMTNMDSEDTATYYCTRRVPSRVMTTSGYFDVWGQGTTVTVSSGGGGSGGGGSGGGGSGSSDIVLTQSPDSLAVSLGERATINCRASQSVSTSTYSYMHWYQQKPGQPPKLLIKYASNLESGVPARFSGSGSETDFTLTIHSMEPEDFATYYCQHSWENPWTFGGGTKVEIKGDPAAALEHHHHHH

SEQ ID NO: 22 - protein, 4 aa, Artificial Sequence
  Description of Artificial Sequence: Synthetic peptide
IEPD

SEQ ID NO: 23 - protein, 4 aa, Artificial Sequence
  Description of Artificial Sequence: Synthetic peptide
KVPL

SEQ ID NO: 24 - protein, 7 aa, Artificial Sequence
  Description of Artificial Sequence: Synthetic peptide
  MOD_RES (2)..(3): Any amino acid
  MOD_RES (5)..(5): Any amino acid
  MOD_RES (7)..(7): Ser or Gly
EXXYXQX

SEQ ID NO: 25 - protein, 5 aa, Artificial Sequence
  Description of Artificial Sequence: Synthetic peptide
  MOD_RES (3)..(3): Any amino acid
LPXTG

SEQ ID NO: 26 - protein, 5 aa, Artificial Sequence
  Description of Artificial Sequence: Synthetic peptide
NPQTN

SEQ ID NO: 27 - protein, 4 aa, Artificial Sequence
  Description of Artificial Sequence: Synthetic peptide
LLQG

SEQ ID NO: 28 - protein, 5 aa, Artificial Sequence
  Description of Artificial Sequence: Synthetic peptide
LPETG

SEQ ID NO: 29 - protein, 6 aa, Artificial Sequence
  Description of Artificial Sequence: Synthetic peptide
RVRRAS

SEQ ID NO: 30 - protein, 4 aa, Artificial Sequence
  Description of Artificial Sequence: Synthetic peptide
IEPF

SEQ ID NO: 31 - protein, 4 aa, Artificial Sequence
  Description of Artificial Sequence: Synthetic peptide
IIPF

SEQ ID NO: 32 - DNA, 146 bp, Artificial Sequence
  Description of Artificial Sequence: Synthetic polynucleotide
gaattcggtatcgagcctttcagcggttccccaggcggcggctccgaaggcggcggaggtattgaaccttttagcggtggaggtggctccgaaggcggtggcgcgcccggtagcactagtggtattataccttttagcgcggccgc

SEQ ID NO: 33 - DNA, 1407 bp, Artificial Sequence
  Description of Artificial Sequence: Synthetic polynucleotide
ggtaccgccgccaccatggactggacctggaggattctcttcttggtggcagcagccacaggagcccactcccagatcgtgctgagccagagccccgccatcctgagcgccagccccggcgagaaggtgaccatgacctgcagggccagcagcagcgtgagctacatccactggttccagcagaagcccggcagcagccccaagccctggatctacgccaccagcaacctggccagcggcgtgcccgtgaggttcagcggcagcggcagcggcaccagctacagcctgaccatcagcagggtggaggccgaggacgccgccacctactactgccagcagtggaccagcaacccccccaccttcggcggcggcaccaagctggagatcaagaggaccgtggccgcccccagcgtgttcatcttcccaccatctgacgagcagctgaagagcggcaccgccagcgtggtgtgcctgctgaacaacttctaccccagggaggccaaggtgcagtggaaggtggacaacgccctgcagagcggcaacagccaggagagcgtgaccgagcaggacagcaaggacagcacctacagcctgagcagcaccctgaccctgagcaaggccgactacgagaagcacaaggtgtacgcctgcgaggtgacccaccagggcctgagcagccccgtgaccaagagcttcaacaggggcgagtgcggtggaggtggatcagaattcggtatcgagcctttcagcggttccccaggcggcggctccgaaggcggcggaggtattgaaccttttagcggtggaggtggctccgaaggcggtggcgcgcccggtagcactagtggtattataccttttagcgcggccgcacctggcggaggcccaaaggctgtgctgaaacttgagcccccgtggatcaacgtgctccaggaggactctgtgactctgacatgccagggggctcgcagccctgagagcgactccattcagtggttccacaatgggaatctcattcccacccacacgcagcccagctacaggttcaaggccaacaacaatgacagcggggagtacacgtgccagactggccagaccagcctcagcgaccctgtgcatctgactgtgctttccgaatggctggtgctccagacccctcacctggagttccaggagggagaaaccatcatgctgaggtgccacagctggaaggacaagcctctggtcaaggtcacattcttccagaatggaaaatcccagaaattctcccgtttggatcccaccttctccatcccacaagcaaaccacagtcacagtggtgattaccactgcacaggaaacataggctacacgctgttctcatccaagcctgtgaccatcactgtccaagtgccctgataatctaga

SEQ ID NO: 34 - protein, 460 aa, Artificial Sequence
  Description of Artificial Sequence: Synthetic polypeptide
MDWTWRILFLVAAATGAHSQIVLSQSPAILSASPGEKVTMTCRASSSVSYIHWFQQKPGSSPKPWIYATSNLASGVPVRFSGSGSGTSYSLTISRVEAEDAATYYCQQWTSNPPTFGGGTKLEIKRTVAAPSVFIFPPSDEQLKSGTASVVCLLNNFYPREAKVQWKVDNALQSGNSQESVTEQDSKDSTYSLSSTLTLSKADYEKHKVYACEVTHQGLSSPVTKSFNRGECGGGGSEFGIEPFSGSPGGGSEGGGGIEPFSGGGGSEGGGAPGSTSGIIPFSAAAPGGGPKAVLKLEPPWINVLQEDSVTLTCQGARSPESDSIQWFHNGNLIPTHTQPSYRFKANNNDSGEYTCQTGQTSLSDPVHLTVLSEWLVLQTPHLEFQEGETIMLRCHSWKDKPLVKVTFFQNGKSQKFSRLDPTFSIPQANHSHSGDYHCTGNIGYTLFSSKPVTITVQVP

SEQ ID NO: 35 - DNA, 1410 bp, Artificial Sequence
  Description of Artificial Sequence: Synthetic polynucleotide
ggtaccgccgccaccatggactggacctggaggattctcttcttggtggcagcagccacaggagcccactccgacatccagatgacccagagccccagcagcctgagcgccagcgtgggcgacagggtgaccatcacctgcagggccagccaggacgtgaacaccgccgtggcctggtatcagcagaagcccggcaaggcccccaagctgctgatctacagcgccagcttcctgtacagcggcgtgcccagcaggttcagcggcagcaggagcggcaccgacttcaccctgaccatcagcagcctgcagcccgaggacttcgccacctactactgccagcagcactacaccaccccccccaccttcggccagggcaccaaggtggagatcaagaggaccgtggccgcccccagcgtgttcatcttcccaccatctgacgagcagctgaagagcggcaccgccagcgtggtgtgcctgctgaacaacttctaccccagggaggccaaggtgcagtggaaggtggacaacgccctgcagagcggcaacagccaggagagcgtgaccgagcaggacagcaaggacagcacctacagcctgagcagcaccctgaccctgagcaaggccgactacgagaagcacaaggtgtacgcctgcgaggtgacccaccagggcctgagcagccccgtgaccaagagcttcaacaggggcgagtgcggtggaggtggatcagaattcggtatcgagcctttcagcggttccccaggcggcggctccgaaggcggcggaggtattgaaccttttagcggtggaggtggctccgaaggcggtggcgcgcccggtagcactagtggtattataccttttagcgcggccgcacctggcggaggcccaaaggctgtgctgaaacttgagcccccgtggatcaacgtgctccaggaggactctgtgactctgacatgccagggggctcgcagccctgagagcgactccattcagtggttccacaatgggaatctcattcccacccacacgcagcccagctacaggttcaaggccaacaacaatgacagcggggagtacacgtgccagactggccagaccagcctcagcgaccctgtgcatctgactgtgctttccgaatggctggtgctccagacccctcacctggagttccaggagggagaaaccatcatgctgaggtgccacagctggaaggacaagcctctggtcaaggtcacattcttccagaatggaaaatcccagaaattctcccgtttggatcccaccttctccatcccacaagcaaaccacagtcacagtggtgattaccactgcacaggaaacataggctacacgctgttctcatccaagcctgtgaccatcactgtccaagtgccctgataatctaga

SEQ ID NO: 36 - protein, 461 aa, Artificial Sequence
  Description of Artificial Sequence: Synthetic polypeptide
MDWTWRILFLVAAATGAHSDIQMTQSPSSLSASVGDRVTITCRASQDVNTAVAWYQQKPGKAPKLLIYSASFLYSGVPSRFSGSRSGTDFTLTISSLQPEDFATYYCQQHYTTPPTFGQGTKVEIKRTVAAPSVFIFPPSDEQLKSGTASVVCLLNNFYPREAKVQWKVDNALQSGNSQESVTEQDSKDSTYSLSSTLTLSKADYEKHKVYACEVTHQGLSSPVTKSFNRGECGGGGSEFGIEPFSGSPGGGSEGGGGIEPFSGGGGSEGGGAPGSTSGIIPFSAAAPGGGPKAVLKLEPPWINVLQEDSVTLTCQGARSPESDSIQWFHNGNLIPTHTQPSYRFKANNNDSGEYTCQTGQTSLSDPVHLTVLSEWLVLQTPHLEFQEGETIMLRCHSWKDKPLVKVTFFQNGKSQKFSRLDPTFSIPQANHSHSGDYHCTGNIGYTLFSSKPVTITVQVP

SEQ ID NO: 37 - DNA, 1527 bp, Artificial Sequence
  Description of Artificial Sequence: Synthetic polynucleotide
ggtaccgccgccaccatggactggacctggaggattctcttcttggtggcagcagccacaggagcccactccgaggtgcagctggtggagagcggcggcggcctggtgcagcccggcggcagcctgaggctgagctgcgccgccagcggcttcaacatcaaggacacctacatccactgggtgaggcaggcccccggcaagggcctggagtgggtggccaggatctaccccaccaacggctacaccaggtacgccgacagcgtgaagggcaggttcaccatcagcgccgacaccagcaagaacaccgcctacctgcagatgaacagcctgagggccgaggacaccgccgtgtactactgcagcaggtggggcggcgacggcttctacgctatggactactggggccagggcaccctggtgaccgtgagcagcgcctccaccaagggcccatcggtcttccccctggcaccctcctccaagagcacctctgggggcacagcggccctgggctgcctggtcaaggactacttccccgagccggtgacggtgtcgtggaactcaggcgccctgaccagcggcgtgcacaccttcccggctgtcctacagtcctcaggactctactccctctcttccgtggtgaccgtgccctccagcagcttgggcacccagacctacatctgcaacgtgaatcacaagcccagcaacaccaaggtggacaagaaagttgagcccaaatcttgtgacactccaccaccttgcccaaggtgcccagcacctgaactcctggggggaccgtcagtcttcctcttccccccaaaacccaaggacaccctcatgatctcccggacccctgaggtcacatgcgtggtggtggacgtgagccacgaagaccctgaggtcaagttcaactggtacgtggacggcgtggaggtgcataatgccaagacaaagccgcgggaggagcagtacaacagcacgtaccgggtggtcagcgtcctcaccgtcctgcaccaggactggctgaatggcaaggagtacaagtgcaaagtctccaacaaagccctgcctgcccccatcgagaaaaccatctccaaagccaaagggcagccccgagaaccacaggtgtacaccctgcccccatcccgggatgagctgaccaagaaccaggtcagcctgacctgcctggtcaaaggcttctatcccagcgacatcgccgtggagtgggagagcaatgggcagccggagaacaactacaagaccacgcctcccgtgctggactccgacggctccttcttcctctactcaaagctcaccgtggacaagagcaggtggcagcaggggaacgtcttctcatgctccgtgatgcatgaggctctgcacaaccactacacgcagaagagcctctccctgtctccgggtaaaggtggaggtggttcacatcatcaccatcatcaccctggcggaggactaaacgacatcttcgaggctcagaaaatcgaatggcacgaaggtccttgataatctaga

SEQ ID NO: 38 - protein, 500 aa, Artificial Sequence
  Description of Artificial Sequence: Synthetic polypeptide
MDWTWRILFLVAAATGAHSEVQLVESGGGLVQPGGSLRLSCAASGFNIKDTYIHWVRQAPGKGLEWVARIYPTNGYTRYADSVKGRFTISADTSKNTAYLQMNSLRAEDTAVYYCSRWGGDGFYAMDYWGQGTLVTVSSASTKGPSVFPLAPSSKSTSGGTAALGCLVKDYFPEPVTVSWNSGALTSGVHTFPAVLQSSGLYSLSSVVTVPSSSLGTQTYICNVNHKPSNTKVDKKVEPKSCDTPPPCPRCPAPELLGGPSVFLFPPKPKDTLMISRTPEVTCVVVDVSHEDPEVKFNWYVDGVEVHNAKTKPREEQYNSTYRVVSVLTVLHQDWLNGKEYKCKVSNKALPAPIEKTISKAKGQPREPQVYTLPPSRDELTKNQVSLTCLVKGFYPSDIAVEWESNGQPENNYKTTPPVLDSDGSFFLYSKLTVDKSRWQQGNVFSCSVMHEALHNHYTQKSLSLSPGKGGGGSHHHHHHPGGGLNDIFEAQKIEWHEGP

SEQ ID NO: 39 - DNA, 726 bp, Artificial Sequence
  Description of Artificial Sequence: Synthetic polynucleotide
ggtaccgccgccaccatggactggacctggaggattctcttcttggtggcagcagccacaggagcccactccgacatccagatgacccagagccccagcagcctgagcgccagcgtgggcgacagggtgaccatcacctgcagggccagccaggacgtgaacaccgccgtggcctggtatcagcagaagcccggcaaggcccccaagctgctgatctacagcgccagcttcctgtacagcggcgtgcccagcaggttcagcggcagcaggagcggcaccgacttcaccctgaccatcagcagcctgcagcccgaggacttcgccacctactactgccagcagcactacaccaccccccccaccttcggccagggcaccaaggtggagatcaagaggaccgtggccgcccccagcgtgttcatcttcccaccatctgacgagcagctgaagagcggcaccgccagcgtggtgtgcctgctgaacaacttctaccccagggaggccaaggtgcagtggaaggtggacaacgccctgcagagcggcaacagccaggagagcgtgaccgagcaggacagcaaggacagcacctacagcctgagcagcaccctgaccctgagcaaggccgactacgagaagcacaaggtgtacgcctgcgaggtgacccaccagggcctgagcagccccgtgaccaagagcttcaacaggggcgagtgctgataatctaga

SEQ ID NO: 40 - protein, 233 aa, Artificial Sequence
  Description of Artificial Sequence: Synthetic polypeptide
MDWTWRILFLVAAATGAHSDIQMTQSPSSLSASVGDRVTITCRASQDVNTAVAWYQQKPGKAPKLLIYSASFLYSGVPSRFSGSRSGTDFTLTISSLQPEDFATYYCQQHYTTPPTFGQGTKVEIKRTVAAPSVFIFPPSDEQLKSGTASVVCLLNNFYPREAKVQWKVDNALQSGNSQESVTEQDSKDSTYSLSSTLTLSKADYEKHKVYACEVTHQGLSSPVTKSFNRGEC

SEQ ID NO: 41 - DNA, 1262 bp, Artificial Sequence
  Description of Artificial Sequence: Synthetic polynucleotide
ccatggataatataaatcgcgctcgcaaaaagcgcgttatcggtggtcatgaagctaaaccgcactcccgtccgtacatggcttacctgatgatctctggtccaagcggttcgaaacgttgcggtggtttcctgatccaggacgacttcgttctgaccgctgctcactgctggggttcctccatcaacgttaccctgggtgctcacaacatcaaagaacaggaaccgacccagcagttcatcccggttaaacgtgctatcccgcacccggcttacaacccgaaaaacttctccaacgacatcatgctgctgcagctggaacagaaagctaaacagacccaggctgttcagccgctgcgtctgccgtccaacaaagctcaggttaaaccgggtcagacctgctccgttgctggttggggtcagaccgctccgctgggtaaacactcccacactctgcaggaagttaaaatgaccgttcaggaagatcgtaaatgcgaatccgacctgcgtcactactacgactccaccatcgaactgtgcgttggtgatccggaaatcaaaaaaacctccttcaaaggtgactccggtggtccgctggtttgcaacaaagttgctcagggtatcgtttcctacggtcgtaccaacggtatgccgccgatcgcttacaccaaagtttcctccttcgttcactggatcgaaaaaactatggaacgttacaccggtcctggtggcggcggttctggtgctagcggtggtcctggcgagctcgaaagatccgttttaacagttccatctacagatatagaaaaagaaatccttgatttagctgctgctacagaaagattaaatttaactgatgcattaaactcaaatccagctggtaatttatatgattggcgttcttctaactcatacccttggactcaaaagctcaatttacacttaacaattacagctactggacaaaaatatagaatcttagctagcaaaattgttgattttaatatttattcaaataattttaataatctagtgaaattagaacagtccttaggtgatggagtaaaagatcattatgttgatataagtttagatgctggacaatatgttcttgtaatgaaagctaattcatcatatagtggaaattacccttattcaatattatttcaaaaatttaagcttgaaggtaagcctatccctaaccctctcctcggtcttgattctacgcgtgcggccgcactcgagcaccaccaccaccaccac

SEQ ID NO: 42 - protein, 420 aa, Artificial Sequence
  Description of Artificial Sequence: Synthetic polypeptide
MDNINRARKKRVIGGHEAKPHSRPYMAYLMISGPSGSKRCGGFLIQDDFVLTAAHCWGSSINVTLGAHNIKEQEPTQQFIPVKRAIPHPAYNPKNFSNDIMLLQLEQKAKQTQAVQPLRLPSNKAQVKPGQTCSVAGWGQTAPLGKHSHTLQEVKMTVQEDRKCESDLRHYYDSTIELCVGDPEIKKTSFKGDSGGPLVCNKVAQGIVSYGRTNGMPPIAYTKVSSFVHWIEKTMERYTGPGGGGSGASGGPGELERSVLTVPSTDIEKEILDLAAATERLNLTDALNSNPAGNLYDWRSSNSYPWTQKLNLHLTITATGQKYRILASKIVDFNIYSNNFNNLVKLEQSLGDGVKDHYVDISLDAGQYVLVMKANSSYSGNYPYSILFQKFKLEGKPIPNPLLGLDSTRAAALEHHHHHH

SEQ ID NO: 43 - DNA, 1938 bp, Artificial Sequence
  Description of Artificial Sequence: Synthetic polynucleotide
ggtaccgccgccaccatggactggacctggaggattctcttcttggtggcagcagccacaggagcccactccgcagcgaattctcaggtgcagctggtccagtctggcgccgaggtcaagaaacctggcgcctccgtgaaagtcagctgcaaggccagcggctacaccttcaccagctacaacatgcactgggtccggcagccccctggcaagggcctggaatggatcggcgccatctaccccggcaacggcgacacctcctacaaccagaagttcaagggcagagtcaccatcaccgccgacaagagcaccagcaccgcctacatggaactgagcagcctgcggagcgaggacaccgccgtgtactactgcgccagaagcacctactacggcggcgactggtacttcaacgtgtggggccagggcaccaccgtgaccgtgtccggtggcggcggcagcggcggcggcggcagcggcggtggctcgagccagatcgtgctgacccagagccccgccaccctgtctctgagccctggcgagagagccaccctgagctgtagagccagcagcagcgtgtcctacatccactggttccagcagaagcccggcaaggcccccaagccctggatctacgccaccagcaacctggccagcggcgtgcccgacagattttctggcagcggcagcggcaccgactacaccctgaagatcagccgggtggaagccgaggacgtgggcacctactactgccagcagtggaccagcaacccccccaccttcggccagggcaccaagctggaaatcaagcgcaccgtggccggtgcggccgcaggaccatctggagcctccaccaagggcccatcggtcttccccctggcaccctcctccaagagcacctctgggggcacagcggccctgggctgcctggtcaaggactacttccccgagccggtgacggtgtcgtggaactcaggcgccctgaccagcggcgtgcacaccttcccggctgtcctacagtcctcaggactctactccctctcttccgtggtgaccgtgccctccagcagcttgggcacccagacctacatctgcaacgtgaatcacaagcccagcaacaccaaggtggacaagaaagttgagcccaaatcttgtgacaaaactcacacatgcccaccgtgcccagcacctgaactcctggggggaccgtcagtcttcctcttccccccaaaacccaaggacaccctcatgatctcccggacccctgaggtcacatgcgtggtggtggacgtgagccacgaagaccctgaggtcaagttcaactggtacgtggacggcgtggaggtgcataatgccaagacaaagccgcgggaggagcagtacaacagcacgtaccgggtggtcagcgtcctcaccgtcctgcaccaggactggctgaatggcaaggagtacaagtgcaaagtctccaacaaagccctgcctgcccccatcgagaaaaccatctccaaagccaaagggcagccccgagaaccacaggtgtacaccctgcccccatcccgggatgagctgaccaagaaccaggtcagcctgacctgcctggtcaaaggcttctatcccagcgacatcgccgtggagtgggagagcaatgggcagccggagaacaactacaagaccacgcctcccgtgctggactccgacggctccttcttcctctactcaaagctcaccgtggacaagagcaggtggcagcaggggaacgtcttctcatgctccgtgatgcatgaggctctgcacaaccactacacgcagaagagcctctccctgtctccgggtaaaggtggaggtggttcacatcatcaccatcatcaccctggcggaggactaaacgacatcttcgaggctcagaaaatcgaatggcacgaaggtccttgataatctaga

SEQ ID NO: 44 - protein, 637 aa, Artificial Sequence
  Description of Artificial Sequence: Synthetic polypeptide
MDWTWRILFLVAAATGAHSAANSQVQLVQSGAEVKKPGASVKVSCKASGYTFTSYNMHWVRQPPGKGLEWIGAIYPGNGDTSYNQKFKGRVTITADKSTSTAYMELSSLRSEDTAVYYCARSTYYGGDWYFNVWGQGTTVTVSGGGGSGGGGSGGGSSQIVLTQSPATLSLSPGERATLSCRASSSVSYIHWFQQKPGKAPKPWIYATSNLASGVPDRFSGSGSGTDYTLKISRVEAEDVGTYYCQQWTSNPPTFGQGTKLEIKRTVAGAAAGPSGASTKGPSVFPLAPSSKSTSGGTAALGCLVKDYFPEPVTVSWNSGALTSGVHTFPAVLQSSGLYSLSSVVTVPSSSLGTQTYICNVNHKPSNTKVDKKVEPKSCDKTHTCPPCPAPELLGGPSVFLFPPKPKDTLMISRTPEVTCVVVDVSHEDPEVKFNWYVDGVEVHNAKTKPREEQYNSTYRVVSVLTVLHQDWLNGKEYKCKVSNKALPAPIEKTISKAKGQPREPQVYTLPPSRDELTKNQVSLTCLVKGFYPSDIAVEWESNGQPENNYKTTPPVLDSDGSFFLYSKLTVDKSRWQQGNVFSCSVMHEALHNHYTQKSLSLSPGKGGGGSHHHHHHPGGGLNDIFEAQKIEWHEGP

SEQ ID NO: 45 - DNA, 1968 bp, Artificial Sequence
  Description of Artificial Sequence: Synthetic polynucleotide
ggtaccgccgccaccatggactggacctggaggattctcttcttggtggcagcagccacaggagcccactccgcagcgaattctcaggtgcagctggtccagtccggcgcggaagtgaaaaaaccgggctcctccgtgaaaatctcctgcaaagcgtccggctacgcgttctcctcctactggatgaactgggtgcgccaggcgccgggccagggcctggaatggatcggccagatctggccgggcgatggcgataccaactacaacggcaaattcaaaggccgcgtgaccctgaccgcggatgaatccacctccaccgcgtacatggaactgtcctccctgcgctccgaagataccgcggtgtacttctgcgcgcgccgcgaaaccaccaccgtgggccgctattactatgcgatggattactggggccagggcaccacggtgaccgtgtcctccggaggcggtggcagcggtggaggtggcagcggcggcgggggtagcgggagctccgatatcctgctgacccagagcccggattccctggccgtgtccctgggcgagcgcgcaaccatcaactgcaaagcgtcccagagcgtggattacgacggcgatagctacctgaactggtaccagcagaaaccgggccagccgccgaaactgctgatctacgatgcgagcaacctggtgtccggcatcccgagccgcttctccggtagtggcagcggcaccgacttcacgctgaccatcagcagtctgcagccggaagatgtcgccacctaccactgccagcagagcaccgaagacccgtggaccttcggccagggcaccaagctggagatcaagcgcggtggtgcggccgcaggaccatctggagcctccaccaagggcccatcggtcttccccctggcaccctcctccaagagcacctctgggggcacagcggccctgggctgcctggtcaaggactacttccccgagccggtgacggtgtcgtggaactcaggcgccctgaccagcggcgtgcacaccttcccggctgtcctacagtcctcaggactctactccctctcttccgtggtgaccgtgccctccagcagcttgggcacccagacctacatctgcaacgtgaatcacaagcccagcaacaccaaggtggacaagaaagttgagcccaaatcttgtgacaaaactcacacatgcccaccgtgcccagcacctgaactcctggggggaccgtcagtcttcctcttccccccaaaacccaaggacaccctcatgatctcccggacccctgaggtcacatgcgtggtggtggacgtgagccacgaagaccctgaggtcaagttcaactggtacgtggacggcgtggaggtgcataatgccaagacaaagccgcgggaggagcagtacaacagcacgtaccgggtggtcagcgtcctcaccgtcctgcaccaggactggctgaatggcaaggagtacaagtgcaaagtctccaacaaagccctgcctgcccccatcgagaaaaccatctccaaagccaaagggcagccccgagaaccacaggtgtacaccctgcccccatcccgggatgagctgaccaagaaccaggtcagcctgacctgcctggtcaaaggcttctatcccagcgacatcgccgtggagtgggagagcaatgggcagccggagaacaactacaagaccacgcctcccgtgctggactccgacggctccttcttcctctactcaaagctcaccgtggacaagagcaggtggcagcaggggaacgtcttctcatgctccgtgatgcatgaggctctgcacaaccactacacgcagaagagcctctccctgtctccgggtaaaggtggaggtggttcacatcatcaccatcatcaccctggcggaggactaaacgacatcttcgaggctcagaaaatcgaatggcacgaaggtccttgataatctaga

SEQ ID NO: 46 - protein, 647 aa, Artificial Sequence
  Description of Artificial Sequence: Synthetic polypeptide
MDWTWRILFLVAAATGAHSAANSQVQLVQSGAEVKKPGSSVKISCKASGYAFSSYWMNWVRQAPGQGLEWIGQIWPGDGDTNYNGKFKGRVTLTADESTSTAYMELSSLRSEDTAVYFCARRETTTVGRYYYAMDYWGQGTTVTVSSGGGGSGGGGSGGGGSGSSDILLTQSPDSLAVSLGERATINCKASQSVDYDGDSYLNWYQQKPGQPPKLLIYDASNLVSGIPSRFSGSGSGTDFTLTISSLQPEDVATYHCQQSTEDPWTFGQGTKLEIKRGGAAAGPSGASTKGPSVFPLAPSSKSTSGGTAALGCLVKDYFPEPVTVSWNSGALTSGVHTFPAVLQSSGLYSLSSVVTVPSSSLGTQTYICNVNHKPSNTKVDKKVEPKSCDKTHTCPPCPAPELLGGPSVFLFPPKPKDTLMISRTPEVTCVVVDVSHEDPEVKFNWYVDGVEVHNAKTKPREEQYNSTYRVVSVLTVLHQDWLNGKEYKCKVSNKALPAPIEKTISKAKGQPREPQVYTLPPSRDELTKNQVSLTCLVKGFYPSDIAVEWESNGQPENNYKTTPPVLDSDGSFFLYSKLTVDKSRWQQGNVFSCSVMHEALHNHYTQKSLSLSPGKGGGGSHHHHHHPGGGLNDIFEAQKIEWHEGP

SEQ ID NO: 47 - DNA, 1152 bp, Artificial Sequence
  Description of Artificial Sequence: Synthetic polynucleotide
ggtaccgccgccaccatggactggacctggaggattctcttcttggtggcagcagccacaggagcccactccgcagcgaattctgaaggatctaccgtggccgcccccagcgtgttcatcttcccaccatctgacgagcagctgaagagcggcaccgccagcgtggtgtgcctgctgaacaacttctaccccagggaggccaaggtgcagtggaaggtggacaacgccctgcagagcggcaacagccaggagagcgtgaccgagcaggacagcaaggacagcacctacagcctgagcagcaccctgaccctgagcaaggccgactacgagaagcacaaggtgtacgcctgcgaggtgacccaccagggcctgagcagccccgtgaccaagagcttcaacaggggcgagtgcggtggaggtggatcagaattcggtatcgagcctttcagcggttccccaggcggcggctccgaaggcggcggaggtattgaaccttttagcggtggaggtggctccgaaggcggtggcgcgcccggtagcactagtggtattataccttttagcgcggccgcacctggcggaggcccaaaggctgtgctgaaacttgagcccccgtggatcaacgtgctccaggaggactctgtgactctgacatgccagggggctcgcagccctgagagcgactccattcagtggttccacaatgggaatctcattcccacccacacgcagcccagctacaggttcaaggccaacaacaatgacagcggggagtacacgtgccagactggccagaccagcctcagcgaccctgtgcatctgactgtgctttccgaatggctggtgctccagacccctcacctggagttccaggagggagaaaccatcatgctgaggtgccacagctggaaggacaagcctctggtcaaggtcacattcttccagaatggaaaatcccagaaattctcccgtttggatcccaccttctccatcccacaagcaaaccacagtcacagtggtgattaccactgcacaggaaacataggctacacgctgttctcatccaagcctgtgaccatcactgtccaagtgcccggtggtggttctggtggaggatggtctcacccacagttcgaaaagtgataatctaga

SEQ ID NO: 48 - protein, 375 aa, Artificial Sequence
  Description of Artificial Sequence: Synthetic polypeptide
MDWTWRILFLVAAATGAHSAANSEGSTVAAPSVFIFPPSDEQLKSGTASVVCLLNNFYPREAKVQWKVDNALQSGNSQESVTEQDSKDSTYSLSSTLTLSKADYEKHKVYACEVTHQGLSSPVTKSFNRGECGGGGSEFGIEPFSGSPGGGSEGGGGIEPFSGGGGSEGGGAPGSTSGIIPFSAAAPGGGPKAVLKLEPPWINVLQEDSVTLTCQGARSPESDSIQWFHNGNLIPTHTQPSYRFKANNNDSGEYTCQTGQTSLSDPVHLTVLSEWLVLQTPHLEFQEGETIMLRCHSWKDKPLVKVTFFQNGKSQKFSRLDPTFSIPQANHSHSGDYHCTGNIGYTLFSSKPVTITVQVPGGGSGGGWSHPQFEK

SEQ ID NO: 49 - DNA, 2367 bp, Artificial Sequence
  Description of Artificial Sequence: Synthetic polynucleotide
ggtaccgccgccaccatggactggacctggaggattctcttcttggtggcagcagccacaggagcccactccgcagcgaattctcaggtgcagctggtccagtctggcgccgaggtcaagaaacctggcgcctccgtgaaagtcagctgcaaggccagcggctacaccttcaccagctacaacatgcactgggtccggcagccccctggcaagggcctggaatggatcggcgccatctaccccggcaacggcgacacctcctacaaccagaagttcaagggcagagtcaccatcaccgccgacaagagcaccagcaccgcctacatggaactgagcagcctgcggagcgaggacaccgccgtgtactactgcgccagaagcacctactacggcggcgactggtacttcaacgtgtggggccagggcaccaccgtgaccgtgtccggtggcggcggcagcggcggcggcggcagcggcggtggctcgagccagatcgtgctgacccagagccccgccaccctgtctctgagccctggcgagagagccaccctgagctgtagagccagcagcagcgtgtcctacatccactggttccagcagaagcccggcaaggcccccaagccctggatctacgccaccagcaacctggccagcggcgtgcccgacagattttctggcagcggcagcggcaccgactacaccctgaagatcagccgggtggaagccgaggacgtgggcacctactactgccagcagtggaccagcaacccccccaccttcggccagggcaccaagctggaaatcaagcgcaccgtggccggtgcggccggtggtactcacacatgcccaccgtgcccagcacctgaactcctggggggaccgtcagtcttcctcttccccccaaaacccaaggacaccctcatgatctcccggacccctgaggtcacatgcgtggtggtggacgtgagccacgaagaccctgaggtcaagttcaactggtacgtggacggcgtggaggtgcataatgccaagacaaagccgcgggaggagcagtacaacagcacgtaccgggtggtcagcgtcctcaccgtcctgcaccaggactggctgaatggcaaggagtacaagtgcaaagtctccaacaaagccctgcctgcccccatcgagaaaaccatctccaaagccaaagggcagccccgagaaccacaggtgtacaccctgcccccatcccgggatgagctgaccaagaaccaggtcagcctgacctgcctggtcaaaggcttctatcccagcgacatcgccgtggagtgggagagcaatgggcagccggagaacaactacaagaccacgcctcccgtgctggactccgacggctccttcttcctctactcaaagctcaccgtggacaagagcaggtggcagcaggggaacgtcttctcatgctccgtgatgcatgaggctctgcacaaccactacacgcagaagagcctctccctgtctccgggtaaaggtggaggtggttcacatcatcaccatcatcaccctggcggaggactaaacgacatcttcgaggctcagaaaatcgaatggcacgaaggtcctgaattcggcggaggcggctccggcggaggcggcgaatccggcggaggcggctccggaggcggcggctccgaaggcggcggaggtattgaaccttttagcggtggaggtggctccgaaggcggtggcggctccggaggcggcggcgaatccggcggcggcggatctggaggcggcggcgaatccggcgcgcccggtagcactagtggtattataccttttagcgcggccgcacctggcggaggcccaaaggctgtgctgaaacttgagcccccgtggatcaacgtgctccaggaggactctgtgactctgacatgccagggggctcgcagccctgagagcgactccattcagtggttccacaatgggaatctcattcccacccacacgcagcccagctacaggttcaaggccaacaacaatgacagcggggagtacacgtgccagactggccagaccagcctcagcgaccctgtgcatctgactgtgctttccgaatggctggtgctccagacccctcacctggagttccaggagggagaaaccatcatgctgaggtgccacagctggaaggacaagcctctggtcaaggtcacattcttccagaatggaaaatcccagaaattctcccgtttggatcccaccttctccatcccacaagcaaaccacagtcacagtggtgattaccactgcacaggaaacataggctacacgctgttctcatccaagcctgtgaccatcactgtccaagtgccctgataatctaga

SEQ ID NO: 50 - protein, 780 aa, Artificial Sequence
  Description of Artificial Sequence: Synthetic polypeptide
MDWTWRILFLVAAATGAHSAANSQVQLVQSGAEVKKPGASVKVSCKASGYTFTSYNMHWVRQPPGKGLEWIGAIYPGNGDTSYNQKFKGRVTITADKSTSTAYMELSSLRSEDTAVYYCARSTYYGGDWYFNVWGQGTTVTVSGGGGSGGGGSGGGSSQIVLTQSPATLSLSPGERATLSCRASSSVSYIHWFQQKPGKAPKPWIYATSNLASGVPDRFSGSGSGTDYTLKISRVEAEDVGTYYCQQWTSNPPTFGQGTKLEIKRTVAGAAGGTHTCPPCPAPELLGGPSVFLFPPKPKDTLMISRTPEVTCVVVDVSHEDPEVKFNWYVDGVEVHNAKTKPREEQYNSTYRVVSVLTVLHQDWLNGKEYKCKVSNKALPAPIEKTISKAKGQPREPQVYTLPPSRDELTKNQVSLTCLVKGFYPSDIAVEWESNGQPENNYKTTPPVLDSDGSFFLYSKLTVDKSRWQQGNVFSCSVMHEALHNHYTQKSLSLSPGKGGGGSHHHHHHPGGGLNDIFEAQKIEWHEGPEFGGGGSGGGGESGGGGSGGGGSEGGGGIEPFSGGGGSEGGGGSGGGGESGGGGSGGGGESGAPGSTSGIIPFSAAAPGGGPKAVLKLEPPWINVLQEDSVTLTCQGARSPESDSIQWFHNGNLIPTHTQPSYRFKANNNDSGEYTCQTGQTSLSDPVHLTVLSEWLVLQTPHLEFQEGETIMLRCHSWKDKPLVKVTFFQNGKSQKFSRLDPTFSIPQANHSHSGDYHCTGNIGYTLFSSKPVTITVQVP

SEQ ID NO: 51 - DNA, 2397 bp, Artificial Sequence
  Description of Artificial Sequence: Synthetic polynucleotide
ggtaccgccgccaccatggactggacctggaggattctcttcttggtggcagcagccacaggagcccactccgcagcgaattctcaggtgcagctggtccagtccggcgcggaagtgaaaaaaccgggctcctccgtgaaaatctcctgcaaagcgtccggctacgcgttctcctcctactggatgaactgggtgcgccaggcgccgggccagggcctggaatggatcggccagatctggccgggcgatggcgataccaactacaacggcaaattcaaaggccgcgtgaccctgaccgcggatgaatccacctccaccgcgtacatggaactgtcctccctgcgctccgaagataccgcggtgtacttctgcgcgcgccgcgaaaccaccaccgtgggccgctattactatgcgatggattactggggccagggcaccacggtgaccgtgtcctccggaggcggtggcagcggtggaggtggcagcggcggcgggggtagcgggagctccgatatcctgctgacccagagcccggattccctggccgtgtccctgggcgagcgcgcaaccatcaactgcaaagcgtcccagagcgtggattacgacggcgatagctacctgaactggtaccagcagaaaccgggccagccgccgaaactgctgatctacgatgcgagcaacctggtgtccggcatcccgagccgcttctccggtagtggcagcggcaccgacttcacgctgaccatcagcagtctgcagccggaagatgtcgccacctaccactgccagcagagcaccgaagacccgtggaccttcggccagggcaccaagctggagatcaagcgcggtggtgcggccggtggtactcacacatgcccaccgtgcccagcacctgaactcctggggggaccgtcagtcttcctcttccccccaaaacccaaggacaccctcatgatctcccggacccctgaggtcacatgcgtggtggtggacgtgagccacgaagaccctgaggtcaagttcaactggtacgtggacggcgtggaggtgcataatgccaagacaaagccgcgggaggagcagtacaacagcacgtaccgggtggtcagcgtcctcaccgtcctgcaccaggactggctgaatggcaaggagtacaagtgcaaagtctccaacaaagccctgcctgcccccatcgagaaaaccatctccaaagccaaagggcagccccgagaaccacaggtgtacaccctgcccccatcccgggatgagctgaccaagaaccaggtcagcctgacctgcctggtcaaaggcttctatcccagcgacatcgccgtggagtgggagagcaatgggcagccggagaacaactacaagaccacgcctcccgtgctggactccgacggctccttcttcctctactcaaagctcaccgtggacaagagcaggtggcagcaggggaacgtcttctcatgctccgtgatgcatgaggctctgcacaaccactacacgcagaagagcctctccctgtctccgggtaaaggtggaggtggttcacatcatcaccatcatcaccctggcggaggactaaacgacatcttcgaggctcagaaaatcgaatggcacgaaggtcctgaattcggcggaggcggctccggcggaggcggcgaatccggcggaggcggctccggaggcggcggctccgaaggcggcggaggtattgaaccttttagcggtggaggtggctccgaaggcggtggcggctccggaggcggcggcgaatccggcggcggcggatctggaggcggcggcgaatccggcgcgcccggtagcactagtggtattataccttttagcgcggccgcacctggcggaggcccaaaggctgtgctgaaacttgagcccccgtggatcaacgtgctccaggaggactctgtgactctgacatgccagggggctcgcagccctgagagcgactccattcagtggttccacaatgggaatctcattcccacccacacgcagcccagctacaggttcaaggccaacaacaatgacagcggggagtacacgtgccagactggccagaccagcctcagcgaccctgtgcatctgactgtgctttccgaatggctggtgctccagacccctcacctggagttccaggagggagaaaccatcatgctgaggtgccacagctggaaggacaagcctctggtcaaggtcacattcttccagaatggaaaatcccagaaattctcccgtttggatcccaccttctccatcccacaagcaaaccacagtcacagtggtgattaccactgcacaggaaacataggctacacgctgttctcatccaagcctgtgaccatcactgtccaagtgccctgataatctaga

SEQ ID NO: 52 - protein, 790 aa, Artificial Sequence
  Description of Artificial Sequence: Synthetic polypeptide
MDWTWRILFLVAAATGAHSAANSQVQLVQSGAEVKKPGSSVKISCKASGYAFSSYWMNWVRQAPGQGLEWIGQIWPGDGDTNYNGKFKGRVTLTADESTSTAYMELSSLRSEDTAVYFCARRETTTVGRYYYAMDYWGQGTTVTVSSGGGGSGGGGSGGGGSGSSDILLTQSPDSLAVSLGERATINCKASQSVDYDGDSYLNWYQQKPGQPPKLLIYDASNLVSGIPSRFSGSGSGTDFTLTISSLQPEDVATYHCQQSTEDPWTFGQGTKLEIKRGGAAGGTHTCPPCPAPELLGGPSVFLFPPKPKDTLMISRTPEVTCVVVDVSHEDPEVKFNWYVDGVEVHNAKTKPREEQYNSTYRVVSVLTVLHQDWLNGKEYKCKVSNKALPAPIEKTISKAKGQPREPQVYTLPPSRDELTKNQVSLTCLVKGFYPSDIAVEWESNGQPENNYKTTPPVLDSDGSFFLYSKLTVDKSRWQQGNVFSCSVMHEALHNHYTQKSLSLSPGKGGGGSHHHHHHPGGGLNDIFEAQKIEWHEGPEFGGGGSGGGGESGGGGSGGGGSEGGGGIEPFSGGGGSEGGGGSGGGGESGGGGSGGGGESGAPGSTSGIIPFSAAAPGGGPKAVLKLEPPWINVLQEDSVTLTCQGARSPESDSIQWFHNGNLIPTHTQPSYRFKANNNDSGEYTCQTGQTSLSDPVHLTVLSEWLVLQTPHLEFQEGETIMLRCHSWKDKPLVKVTFFQNGKSQKFSRLDPTFSIPQANHSHSGDYHCTGNIGYTLFSSKPVTITVQVP

SEQ ID NO: 53 - DNA, 1992 bp, Artificial Sequence
  Description of Artificial Sequence: Synthetic polynucleotide
ggtaccgccgccaccatggactggacctggaggattctcttcttggtggcagcagccacaggagcccactccgcagcgaattctgctgctgctacagaaagattaaatttagctgatgcattaaactcaaatccagctggtaatttatatgattggcgttcttctaactcatacccttggactcaaaagctcaatttacacttaacaattacagctactggacaaaaatatagaatcttagctagcaaaattgttgattttaatatttattcaaataattttaataatctagtgaaattagaacagtccttaggtgatggagtaaaagatcattatgttgatataagtttagatgctggacaatatgttcttgtaatgaaagctaattcagcatatagtggaaattacccttattcaatattatttcaaaaatttaagggtggtcctgcggccggtggtactcacacatgcccaccgtgcccagcacctgaactcctggggggaccgtcagtcttcctcttccccccaaaacccaaggacaccctcatgatctcccggacccctgaggtcacatgcgtggtggtggacgtgagccacgaagaccctgaggtcaagttcaactggtacgtggacggcgtggaggtgcataatgccaagacaaagccgcgggaggagcagtacaacagcacgtaccgggtggtcagcgtcctcaccgtcctgcaccaggactggctgaatggcaaggagtacaagtgcaaagtctccaacaaagccctgcctgcccccatcgagaaaaccatctccaaagccaaagggcagccccgagaaccacaggtgtacaccctgcccccatcccgggatgagctgaccaagaaccaggtcagcctgacctgcctggtcaaaggcttctatcccagcgacatcgccgtggagtgggagagcaatgggcagccggagaacaactacaagaccacgcctcccgtgctggactccgacggctccttcttcctctactcaaagctcaccgtggacaagagcaggtggcagcaggggaacgtcttctcatgctccgtgatgcatgaggctctgcacaaccactacacgcagaagagcctctccctgtctccgggtaaaggtggaggtggttcacatcatcaccatcatcaccctggcggaggactaaacgacatcttcgaggctcagaaaatcgaatggcacgaaggtcctgaattcggcggaggcggctccggcggaggcggcgaatccggcggaggcggctccggaggcggcggctccgaaggcggcggaggtattgaaccttttagcggtggaggtggctccgaaggcggtggcggctccggaggcggcggcgaatccggcggcggcggatctggaggcggcggcgaatccggcgcgcccggtagcactagtggtattataccttttagcgcggccgcacctggcggaggcccaaaggctgtgctgaaacttgagcccccgtggatcaacgtgctccaggaggactctgtgactctgacatgccagggggctcgcagccctgagagcgactccattcagtggttccacaatgggaatctcattcccacccacacgcagcccagctacaggttcaaggccaacaacaatgacagcggggagtacacgtgccagactggccagaccagcctcagcgaccctgtgcatctgactgtgctttccgaatggctggtgctccagacccctcacctggagttccaggagggagaaaccatcatgctgaggtgccacagctggaaggacaagcctctggtcaaggtcacattcttccagaatggaaaatcccagaaattctcccgtttggatcccaccttctccatcccacaagcaaaccacagtcacagtggtgattaccactgcacaggaaacataggctacacgctgttctcatccaagcctgtgaccatcactgtccaagtgccctgataatctaga

SEQ ID NO: 54 - protein, 655 aa, Artificial Sequence
  Description of Artificial Sequence: Synthetic polypeptide
MDWTWRILFLVAAATGAHSAANSAAATERLNLADALNSNPAGNLYDWRSSNSYPWTQKLNLHLTITATGQKYRILASKIVDFNIYSNNFNNLVKLEQSLGDGVKDHYVDISLDAGQYVLVMKANSAYSGNYPYSILFQKFKGGPAAGGTHTCPPCPAPELLGGPSVFLFPPKPKDTLMISRTPEVTCVVVDVSHEDPEVKFNWYVDGVEVHNAKTKPREEQYNSTYRVVSVLTVLHQDWLNGKEYKCKVSNKALPAPIEKTISKAKGQPREPQVYTLPPSRDELTKNQVSLTCLVKGFYPSDIAVEWESNGQPENNYKTTPPVLDSDGSFFLYSKLTVDKSRWQQGNVFSCSVMHEALHNHYTQKSLSLSPGKGGGGSHHHHHHPGGGLNDIFEAQKIEWHEGPEFGGGGSGGGGESGGGGSGGGGSEGGGGIEPFSGGGGSEGGGGSGGGGESGGGGSGGGGESGAPGSTSGIIPFSAAAPGGGPKAVLKLEPPWINVLQEDSVTLTCQGARSPESDSIQWFHNGNLIPTHTQPSYRFKANNNDSGEYTCQTGQTSLSDPVHLTVLSEWLVLQTPHLEFQEGETIMLRCHSWKDKPLVKVTFFQNGKSQKFSRLDPTFSIPQANHSHSGDYHCTGNIGYTLFSSKPVTITVQVP

SEQ ID NO: 55 - DNA, 2184 bp, Artificial Sequence
  Description of Artificial Sequence: Synthetic polynucleotide
ggtaccgccgccaccatggactggacctggaggattctcttcttggtggcagcagccacaggagcccactccgcagcgaattctaaagagattacgaatgccttggaaacctggggtgccttgggtcaggacatcaacttggacattcctagttttcaaatgagtgatgatattgacgatataaaatgggaaaaaacttcagacaagaaaaagattgcacaattcagaaaagagaaagagactttcaaggaaaaagatacatataagctatttaaaaatggaactctgaaaattaagcatctgaagaccgatgatcaggatatctacaaggtatcaatatatgatacaaaaggaaaaaatgtgttggaaaaaatatttgatttgaagattcaagagagggtctcaaaaccaaagatctcctggacttgtatcaacacaaccctgacctgtgaggtaatgaatggaactgaccccgaattaaacctgtatcaagatgggaaacatctaaaactttctcagagggtcatcacacacaagtggaccaccagcctgagtgcaaaattcaagtgcacagcagggaacaaagtcagcaaggaatccagtgtcgagcctgtcagctgtccagagaaaggtctggacgcggccggtggtactcacacatgcccaccgtgcccagcacctgaactcctggggggaccgtcagtcttcctcttccccccaaaacccaaggacaccctcatgatctcccggacccctgaggtcacatgcgtggtggtggacgtgagccacgaagaccctgaggtcaagttcaactggtacgtggacggcgtggaggtgcataatgccaagacaaagccgcgggaggagcagtacaacagcacgtaccgggtggtcagcgtcctcaccgtcctgcaccaggactggctgaatggcaaggagtacaagtgcaaagtctccaacaaagccctgcctgcccccatcgagaaaaccatctccaaagccaaagggcagccccgagaaccacaggtgtacaccctgcccccatcccgggatgagctgaccaagaaccaggtcagcctgacctgcctggtcaaaggcttctatcccagcgacatcgccgtggagtgggagagcaatgggcagccggagaacaactacaagaccacgcctcccgtgctggactccgacggctccttcttcctctactcaaagctcaccgtggacaagagcaggtggcagcaggggaacgtcttctcatgctccgtgatgcatgaggctctgcacaaccactacacgcagaagagcctctccctgtctccgggtaaaggtggaggtggttcacatcatcaccatcatcaccctggcggaggactaaacgacatcttcgaggctcagaaaatcgaatggcacgaaggtcctgaattcggcggaggcggctccggcggaggcggcgaatccggcggaggcggctccggaggcggcggctccgaaggcggcggaggtattgaaccttttagcggtggaggtggctccgaaggcggtggcggctccggaggcggcggcgaatccggcggcggcggatctggaggcggcggcgaatccggcgcgcccggtagcactagtggtattataccttttagcgcggccgcacctggcggaggcccaaaggctgtgctgaaacttgagcccccgtggatcaacgtgctccaggaggactctgtgactctgacatgccagggggctcgcagccctgagagcgactccattcagtggttccacaatgggaatctcattcccacccacacgcagcccagctacaggttcaaggccaacaacaatgacagcggggagtacacgtgccagactggccagaccagcctcagcgaccctgtgcatctgactgtgctttccgaatggctggtgctccagacccctcacctggagttccaggagggagaaaccatcatgctgaggtgccacagctggaaggacaagcctctggtcaaggtcacattcttccagaatggaaaatcccagaaattctcccgtttggatcccaccttctccatcccacaagcaaaccacagtcacagtggtgattaccactgcacaggaaacataggctacacgctgttctcatccaagcctgtgaccatcactgtccaagtgccctgataatctaga

SEQ ID NO: 56 - protein, 719 aa, Artificial Sequence
  Description of Artificial Sequence: Synthetic polypeptide
MDWTWRILFLVAAATGAHSAANSKEITNALETWGALGQDINLDIPSFQMSDDIDDIKWEKTSDKKKIAQFRKEKETFKEKDTYKLFKNGTLKIKHLKTDDQDIYKVSIYDTKGKNVLEKIFDLKIQERVSKPKISWTCINTTLTCEVMNGTDPELNLYQDGKHLKLSQRVITHKWTTSLSAKFKCTAGNKVSKESSVEPVSCPEKGLDAAGGTHTCPPCPAPELLGGPSVFLFPPKPKDTLMISRTPEVTCVVVDVSHEDPEVKFNWYVDGVEVHNAKTKPREEQYNSTYRVVSVLTVLHQDWLNGKEYKCKVSNKALPAPIEKTISKAKGQPREPQVYTLPPSRDELTKNQVSLTCLVKGFYPSDIAVEWESNGQPENNYKTTPPVLDSDGSFFLYSKLTVDKSRWQQGNVFSCSVMHEALHNHYTQKSLSLSPGKGGGGSHHHHHHPGGGLNDIFEAQKIEWHEGPEFGGGGSGGGGESGGGGSGGGGSEGGGGIEPFSGGGGSEGGGGSGGGGESGGGGSGGGGESGAPGSTSGIIPFSAAAPGGGPKAVLKLEPPWINVLQEDSVTLTCQGARSPESDSIQWFHNGNLIPTHTQPSYRFKANNNDSGEYTCQTGQTSLSDPVHLTVLSEWLVLQTPHLEFQEGETIMLRCHSWKDKPLVKVTFFQNGKSQKFSRLDPTFSIPQANHSHSGDYHCTGNIGYTLFSSKPVTITVQVP

SEQ ID NO: 57 - DNA, 1989 bp, Artificial Sequence
  Description of Artificial Sequence: Synthetic polynucleotide
ggtaccgccgccaccatggactggacctggaggattctcttcttggtggcagcagccacaggagcccactccgcagcgaattctctgggcaagaagctgctggaggccgccagggccggccaggacgacgaggttaggatcctgatggccaacggcgccgacgtgaacgccaaggacgagtacggcctgacccccctgtacctggccaccgcccacggccacctggagatcgtggaggtgctgctgaagaatggagcagatgttaatgctgtggacgccatcggcttcacccccctgcacctggccgccttcatcggacatcttgaaattgccgaagtcttgcttaaacacggtgctgacgtcaatgcacaggacaagttcggcaagaccgccttcgacatcagcatcggcaacggcaacgaggacctggccgagatcctgcaggcggccggtggtactcacacatgcccaccgtgcccagcacctgaactcctggggggaccgtcagtcttcctcttccccccaaaacccaaggacaccctcatgatctcccggacccctgaggtcacatgcgtggtggtggacgtgagccacgaagaccctgaggtcaagttcaactggtacgtggacggcgtggaggtgcataatgccaagacaaagccgcgggaggagcagtacaacagcacgtaccgggtggtcagcgtcctcaccgtcctgcaccaggactggctgaatggcaaggagtacaagtgcaaagtctccaacaaagccctgcctgcccccatcgagaaaaccatctccaaagccaaagggcagccccgagaaccacaggtgtacaccctgcccccatcccgggatgagctgaccaagaaccaggtcagcctgacctgcctggtcaaaggcttctatcccagcgacatcgccgtggagtgggagagcaatgggcagccggagaacaactacaagaccacgcctcccgtgctggactccgacggctccttcttcctctactcaaagctcaccgtggacaagagcaggtggcagcaggggaacgtcttctcatgctccgtgatgcatgaggctctgcacaaccactacacgcagaagagcctctccctgtctccgggtaaaggtggaggtggttcacatcatcaccatcatcaccctggcggaggactaaacgacatcttcgaggctcagaaaatcgaatggcacgaaggtcctgaattcggcggaggcggctccggcggaggcggcgaatccggcggaggcggctccggaggcggcggctccgaaggcggcggaggtattgaaccttttagcggtggaggtggctccgaaggcggtggcggctccggaggcggcggcgaatccggcggcggcggatctggaggcggcggcgaatccggcgcgcccggtagcactagtggtattataccttttagcgcggccgcacctggcggaggcccaaaggctgtgctgaaacttgagcccccgtggatcaacgtgctccaggaggactctgtgactctgacatgccagggggctcgcagccctgagagcgactccattcagtggttccacaatgggaatctcattcccacccacacgcagcccagctacaggttcaaggccaacaacaatgacagcggggagtacacgtgccagactggccagaccagcctcagcgaccctgtgcatctgactgtgctttccgaatggctggtgctccagacccctcacctggagttccaggagggagaaaccatcatgctgaggtgccacagctggaaggacaagcctctggtcaaggtcacattcttccagaatggaaaatcccagaaattctcccgtttggatcccaccttctccatcccacaagcaaaccacagtcacagtggtgattaccactgcacaggaaacataggctacacgctgttctcatccaagcctgtgaccatcactgtccaagtgccctgataatctaga

SEQ ID NO: 58 - protein, 654 aa, Artificial Sequence
  Description of Artificial Sequence: Synthetic polypeptide
MDWTWRILFLVAAATGAHSAANSLGKKLLEAARAGQDDEVRILMANGADVNAKDEYGLTPLYLATAHGHLEIVEVLLKNGADVNAVDAIGFTPLHLAAFIGHLEIAEVLLKHGADVNAQDKFGKTAFDISIGNGNEDLAEILQAAGGTHTCPPCPAPELLGGPSVFLFPPKPKDTLMISRTPEVTCVVVDVSHEDPEVKFNWYVDGVEVHNAKTKPREEQYNSTYRVVSVLTVLHQDWLNGKEYKCKVSNKALPAPIEKTISKAKGQPREPQVYTLPPSRDELTKNQVSLTCLVKGFYPSDIAVEWESNGQPENNYKTTPPVLDSDGSFFLYSKLTVDKSRWQQGNVFSCSVMHEALHNHYTQKSLSLSPGKGGGGSHHHHHHPGGGLNDIFEAQKIEWHEGPEFGGGGSGGGGESGGGGSGGGGSEGGGGIEPFSGGGGSEGGGGSGGGGESGGGGSGGGGESGAPGSTSGIIPFSAAAPGGGPKAVLKLEPPWINVLQEDSVTLTCQGARSPESDSIQWFHNGNLIPTHTQPSYRFKANNNDSGEYTCQTGQTSLSDPVHLTVLSEWLVLQTPHLEFQEGETIMLRCHSWKDKPLVKVTFFQNGKSQKFSRLDPTFSIPQANHSHSGDYHCTGNIGYTLFSSKPVTITVQVP

SEQ ID NO: 59 - DNA, 1151 bp, Artificial Sequence
  Description of Artificial Sequence: Synthetic polynucleotide
ccatggataatataaatcgcgctcgcaaaaagcgcgttatcggtggtcatgaagctaaaccgcactcccgtccgtacatggcttacctgatgatctctggtccaagcggttcgaaacgttgcggtggtttcctgatccaggacgacttcgttctgaccgctgctcactgctggggttcctccatcaacgttaccctgggtgctcacaacatcaaagaacaggaaccgacccagcagttcatcccggttaaacgtgctatcccgcacccggcttacaacccgaaaaacttctccaacgacatcatgctgctgcagctggaacagaaagctaaacagacccaggctgttcagccgctgcgtctgccgtccaacaaagctcaggttaaaccgggtcagacctgctccgttgctggttggggtcagaccgctccgctgggtaaacactcccacactctgcaggaagttaaaatgaccgttcaggaagatcgtaaatgcgaatccgacctgcgtcactactacgactccaccatcgaactgtgcgttggtgatccggaaatcaaaaaaacctccttcaaaggtgactccggtggtccgctggtttgcaacaaagttgctcagggtatcgtttcctacggtcgtaccaacggtatgccgccgatcgcttacaccaaagtttcctccttcgttcactggatcgaaaaaactatggaacgttacaccggtcctggtggcggcggttctggtgctagcggtggttctctgggcaagaagctgctggaggccgccagggccggccaggacgacgaggttaggatcctgatggccaacggcgccgacgtgaacgccaaggacgagtacggcctgacccccctgtacctggccaccgcccacggccacctggagatcgtggaggtgctgctgaagaatggagcagatgttaatgctgtggacgccatcggcttcacccccctgcacctggccgccttcatcggacatcttgaaattgccgaagtcttgcttaaacacggtgctgacgtcaatgcacaggacaagttcggcaagaccgccttcgacatcagcatcggcaacggcaacgaggacctggccgagatcctgcaggcggccgcactcgagcaccaccaccaccaccac

SEQ ID NO: 60 - protein, 383 aa, Artificial Sequence
  Description of Artificial Sequence: Synthetic polypeptide
MDNINRARKKRVIGGHEAKPHSRPYMAYLMISGPSGSKRCGGFLIQDDFVLTAAHCWGSSINVTLGAHNIKEQEPTQQFIPVKRAIPHPAYNPKNFSNDIMLLQLEQKAKQTQAVQPLRLPSNKAQVKPGQTCSVAGWGQTAPLGKHSHTLQEVKMTVQEDRKCESDLRHYYDSTIELCVGDPEIKKTSFKGDSGGPLVCNKVAQGIVSYGRTNGMPPIAYTKVSSFVHWIEKTMERYTGPGGGGSGASGGSLGKKLLEAARAGQDDEVRILMANGADVNAKDEYGLTPLYLATAHGHLEIVEVLLKNGADVNAVDAIGFTPLHLAAFIGHLEIAEVLLKHGADVNAQDKFGKTAFDISIGNGNEDLAEILQAAALEHHHHHH

SEQ ID NO: 61 - DNA, 1488 bp, Artificial Sequence
  Description of Artificial Sequence: Synthetic polynucleotide
ggtaccgccgccaccatggactggacctggaggattctcttcttggtggcagcagccacaggagcccactcccagatcgtgctgagccagagccccgccatcctgagcgccagccccggcgagaaggtgaccatgacctgcagggccagcagcagcgtgagctacatccactggttccagcagaagcccggcagcagccccaagccctggatctacgccaccagcaacctggccagcggcgtgcccgtgaggttcagcggcagcggcagcggcaccagctacagcctgaccatcagcagggtggaggccgaggacgccgccacctactactgccagcagtggaccagcaacccccccaccttcggcggcggcaccaagctggagatcaagaggaccgtggccgcccccagcgtgttcatcttcccaccatctgacgagcagctgaagagcggcaccgccagcgtggtgtgcctgctgaacaacttctaccccagggaggccaaggtgcagtggaaggtggacaacgccctgcagagcggcaacagccaggagagcgtgaccgagcaggacagcaaggacagcacctacagcctgagcagcaccctgaccctgagcaaggccgactacgagaagcacaaggtgtacgcctgcgaggtgacccaccagggcctgagcagccccgtgaccaagagcttcaacaggggcgagtgcggtggaggtggatcagaattcggtatcgagcctttcagcggttccccaggcggcggctccgaaggcggcggaggtattgaaccttttagcggtggaggtggctccgaaggcggtggcgcgcccggtagcactagtggtattataccttttagcgcggccgcaagcggccacgccaagcagaaccagaagagcgtgaacaagcacgacaaggaggccctgcacaggtactacaccggcaacttcaaggagatgaagaacatcaacgccctgaagcacggcaagaacaacctgaggttcaagtacaggggcatgaagacccaggtgctgctgcccggcaacgagtacaggaagtaccagcagaggaggtacaccggcctggacgtgttcttcgtgcaggagaggagggacaagcacgacatcagctacaccgtgggcggcgtgaccaagaccaacaaggccagcggcttcgtgagcgagcccaggctgaacgtggccaaggagaacggcaaggacgccttcgtgaagggctacccctaccacatcaacaaggaggagatcagcctgaaggagctggacttcaagctgaggaagcacctgatcgagaagtacggcctgtacaagaccatcagcaaggagggcagggtgaagatcagcctgaaggacggcagcttctacaacctggacctgaggtacaagctggacttcaagtacatgggcgaggtgatcgacagcaagcagatcaaggacatcgaggttaacctgaagtaataatctaga

SEQ ID NO: 62 - protein, 487 aa, Artificial Sequence
  Description of Artificial Sequence: Synthetic polypeptide
MDWTWRILFLVAAATGAHSQIVLSQSPAILSASPGEKVTMTCRASSSVSYIHWFQQKPGSSPKPWIYATSNLASGVPVRFSGSGSGTSYSLTISRVEAEDAATYYCQQWTSNPPTFGGGTKLEIKRTVAAPSVFIFPPSDEQLKSGTASVVCLLNNFYPREAKVQWKVDNALQSGNSQESVTEQDSKDSTYSLSSTLTLSKADYEKHKVYACEVTHQGLSSPVTKSFNRGECGGGGSEFGIEPFSGSPGGGSEGGGGIEPFSGGGGSEGGGAPGSTSGIIPFSAAASGHAKQNQKSVNKHDKEALHRYYTGNFKEMKNINALKHGKNNLRFKYRGMKTQVLLPGNEYRKYQQRRYTGLDVFFVQERRDKHDISYTVGGVTKTNKASGFVSEPRLNVAKENGKDAFVKGYPYHINKEEISLKELDFKLRKHLIEKYGLYKTISKEGRVKISLKDGSFYNLDLRYKLDFKYMGEVIDSKQIKDIEVNLK

SEQ ID NO: 63 - DNA, 1323 bp, Artificial Sequence
  Description of Artificial Sequence: Synthetic polynucleotide
ggtaccgccgccaccatggactggacctggaggattctcttcttggtggcagcagccacaggagcccactcccagatcgtgctgagccagagccccgccatcctgagcgccagccccggcgagaaggtgaccatgacctgcagggccagcagcagcgtgagctacatccactggttccagcagaagcccggcagcagccccaagccctggatctacgccaccagcaacctggccagcggcgtgcccgtgaggttcagcggcagcggcagcggcaccagctacagcctgaccatcagcagggtggaggccgaggacgccgccacctactactgccagcagtggaccagcaacccccccaccttcggcggcggcaccaagctggagatcaagaggaccgtggccgcccccagcgtgttcatcttcccaccatctgacgagcagctgaagagcggcaccgccagcgtggtgtgcctgctgaacaacttctaccccagggaggccaaggtgcagtggaaggtggacaacgccctgcagagcggcaacagccaggagagcgtgaccgagcaggacagcaaggacagcacctacagcctgagcagcaccctgaccctgagcaaggccgactacgagaagcacaaggtgtacgcctgcgaggtgacccaccagggcctgagcagccccgtgaccaagagcttcaacaggggcgagtgcggtggaggtggatcagaattcggtatcgagcctttcagcggttccccaggcggcggctccgaaggcggcggaggtattgaaccttttagcggtggaggtggctccgaaggcggtggcgcgcccggtagcactagtggtattataccttttagcgcggccgcatcccccggggagacgttcagcacgaacgtctccatccatgccatcgcccacgacgaccagacctactccatggacgtcgtctggttgaggttcgacgtgccgacctcgtgtgccgagatgcgaatatacgaatcgtgtctgtatcacccgcagctcccagaatgtctgtccccggccgacgcgccgtgcgccgcgagtacgtggacgtctcgcctggccgtccgcagctacgcggggtgttccagaacaaaccccccaccgcgctgttcggccgaggctcacatggagcccgtcccggggctggcgtggcaggcggcctccgtcaatctggagttccgggacgcgtccccacaacactccggcctgtatctgtgtgtggtgtacgtcaacgaccatattcacgcctggggccacattaccatcagcaccgcggcgcagtaataatctaga

SEQ ID NO: 64 - protein, 432 aa, Artificial Sequence
  Description of Artificial Sequence: Synthetic polypeptide
MDWTWRILFLVAAATGAHSQIVLSQSPAILSASPGEKVTMTCRASSSVSYIHWFQQKPGSSPKPWIYATSNLASGVPVRFSGSGSGTSYSLTISRVEAEDAATYYCQQWTSNPPTFGGGTKLEIKRTVAAPSVFIFPPSDEQLKSGTASVVCLLNNFYPREAKVQWKVDNALQSGNSQESVTEQDSKDSTYSLSSTLTLSKADYEKHKVYACEVTHQGLSSPVTKSFNRGECGGGGSEFGIEPFSGSPGGGSEGGGGIEPFSGGGGSEGGGAPGSTSGIIPFSAAASPGETFSTNVSIHAIAHDDQTYSMDVVWLRFDVPTSCAEMRIYESCLYHPQLPECLSPADAPCAASTWTSRLAVRSYAGCSRTNPPPRCSAEAHMEPVPGLAWQAASVNLEFRDASPQHSGLYLCVVYVNDHIHAWGHITISTAAQ

SEQ ID NO: 65 - DNA, 1245 bp, Artificial Sequence
  Description of Artificial Sequence: Synthetic polynucleotide
ggtaccgccgccaccatggactggacctggaggattctcttcttggtggcagcagccacaggagcccactcccagatcgtgctgagccagagccccgccatcctgagcgccagccccggcgagaaggtgaccatgacctgcagggccagcagcagcgtgagctacatccactggttccagcagaagcccggcagcagccccaagccctggatctacgccaccagcaacctggccagcggcgtgcccgtgaggttcagcggcagcggcagcggcaccagctacagcctgaccatcagcagggtggaggccgaggacgccgccacctactactgccagcagtggaccagcaacccccccaccttcggcggcggcaccaagctggagatcaagaggaccgtggccgcccccagcgtgttcatcttcccaccatctgacgagcagctgaagagcggcaccgccagcgtggtgtgcctgctgaacaacttctaccccagggaggccaaggtgcagtggaaggtggacaacgccctgcagagcggcaacagccaggagagcgtgaccgagcaggacagcaaggacagcacctacagcctgagcagcaccctgaccctgagcaaggccgactacgagaagcacaaggtgtacgcctgcgaggtgacccaccagggcctgagcagccccgtgaccaagagcttcaacaggggcgagtgcggtggaggtggatcagaattcggtatcgagcctttcagcggttccccaggcggcggctccgaaggcggcggaggtattgaaccttttagcggtggaggtggctccgaaggcggtggcgcgcccggtagcactagtggtattataccttttagcgcggccgcactgggcaagaagctgctggaggccgccagggccggccaggacgacgaggttaggatcctgatggccaacggcgccgacgtgaacgccagggacatgtctggctacacccccctgcacctggccgcccacatgggccacctggagatcgtggaggtgctgctgaagaatggagcagatgttaatgctaaagacaactggggcgacacccccctgcacctggccgccatcttcggacatcttgaaattgtcgaagtcttgcttaaaaacggtgctgacgtcaatgcacaggacaagttcggcaagaccgccttcgacatcagcatcgacaacggcaacgaggacctggccgagatcctgcagtaataatctaga

SEQ ID NO: 66 - protein, 406 aa, Artificial Sequence
  Description of Artificial Sequence: Synthetic polypeptide
MDWTWRILFLVAAATGAHSQIVLSQSPAILSASPGEKVTMTCRASSSVSYIHWFQQKPGSSPKPWIYATSNLASGVPVRFSGSGSGTSYSLTISRVEAEDAATYYCQQWTSNPPTFGGGTKLEIKRTVAAPSVFIFPPSDEQLKSGTASVVCLLNNFYPREAKVQWKVDNALQSGNSQESVTEQDSKDSTYSLSSTLTLSKADYEKHKVYACEVTHQGLSSPVTKSFNRGECGGGGSEFGIEPFSGSPGGGSEGGGGIEPFSGGGGSEGGGAPGSTSGIIPFSAAALGKKLLEAARAGQDDEVRILMANGADVNARDMSGYTPLHLAAHMGHLEIVEVLLKNGADVNAKDNWGDTPLHLAAIFGHLEIVEVLLKNGADVNAQDKFGKTAFDISIDNGNEDLAEILQ

SEQ ID NO: 67 - DNA, 1245 bp, Artificial Sequence
  Description of Artificial Sequence: Synthetic polynucleotide
ggtaccgccgccaccatggactggacctggaggattctcttcttggtggcagcagccacaggagcccactcccagatcgtgctgagccagagccccgccatcctgagcgccagccccggcgagaaggtgaccatgacctgcagggccagcagcagcgtgagctacatccactggttccagcagaagcccggcagcagccccaagccctggatctacgccaccagcaacctggccagcggcgtgcccgtgaggttcagcggcagcggcagcggcaccagctacagcctgaccatcagcagggtggaggccgaggacgccgccacctactactgccagcagtggaccagcaacccccccaccttcggcggcggcaccaagctggagatcaagaggaccgtggccgcccccagcgtgttcatcttcccaccatctgacgagcagctgaagagcggcaccgccagcgtggtgtgcctgctgaacaacttctaccccagggaggccaaggtgcagtggaaggtggacaacgccctgcagagcggcaacagccaggagagcgtgaccgagcaggacagcaaggacagcacctacagcctgagcagcaccctgaccctgagcaaggccgactacgagaagcacaaggtgtacgcctgcgaggtgacccaccagggcctgagcagccccgtgaccaagagcttcaacaggggcgagtgcggtggaggtggatcagaattcggtatcgagcctttcagcggttccccaggcggcggctccgaaggcggcggaggtattgaaccttttagcggtggaggtggctccgaaggcggtggcgcgcccggtagcactagtggtattataccttttagcgcggccgcactgggcaagaagctgctggaggccgccagggccggccaggacgacgaggttaggatcctgatggccaacggcgccgacgtgaacgccgcggacaagtctggctacacccccctgcacctggccgcccacattggccacctggagatcgtggaggtgctgctgaagcacggagcagatgttaatgctcatgacagctggggcgacacccccctgcacctggccgccaccttcggacatcttgaaattgtcgaagtcttgcttaaacacggtgctgacgtcaatgcacaggacaagttcggcaagaccgccttcgacatcagcatcgacaacggcaacgaggacctggccgagatcctgcagtaataatctaga

SEQ ID NO: 68 - protein, 406 aa, Artificial Sequence
  Description of Artificial Sequence: Synthetic polypeptide
MDWTWRILFLVAAATGAHSQIVLSQSPAILSASPGEKVTMTCRASSSVSYIHWFQQKPGSSPKPWIYATSNLASGVPVRFSGSGSGTSYSLTISRVEAEDAATYYCQQWTSNPPTFGGGTKLEIKRTVAAPSVFIFPPSDEQLKSGTASVVCLLNNFYPREAKVQWKVDNALQSGNSQESVTEQDSKDSTYSLSSTLTLSKADYEKHKVYACEVTHQGLSSPVTKSFNRGECGGGGSEFGIEPFSGSPGGGSEGGGGIEPFSGGGGSEGGGAPGSTSGIIPFSAAALGKKLLEAARAGQDDEVRILMANGADVNAADKSGYTPLHLAAHIGHLEIVEVLLKHGADVNAHDSWGDTPLHLAATFGHLEIVEVLLKHGADVNAQDKFGKTAFDISIDNGNEDLAEILQ

SEQ ID NO: 69 - DNA, 1344 bp, Artificial Sequence
  Description of Artificial Sequence: Synthetic polynucleotide
ggtaccgccgccaccatggactggacctggaggattctcttcttggtggcagcagccacaggagcccactcccagatcgtgctgagccagagccccgccatcctgagcgccagccccggcgagaaggtgaccatgacctgcagggccagcagcagcgtgagctacatccactggttccagcagaagcccggcagcagccccaagccctggatctacgccaccagcaacctggccagcggcgtgcccgtgaggttcagcggcagcggcagcggcaccagctacagcctgaccatcagcagggtggaggccgaggacgccgccacctactactgccagcagtggaccagcaacccccccaccttcggcggcggcaccaagctggagatcaagaggaccgtggccgcccccagcgtgttcatcttcccaccatctgacgagcagctgaagagcggcaccgccagcgtggtgtgcctgctgaacaacttctaccccagggaggccaaggtgcagtggaaggtggacaacgccctgcagagcggcaacagccaggagagcgtgaccgagcaggacagcaaggacagcacctacagcctgagcagcaccctgaccctgagcaaggccgactacgagaagcacaaggtgtacgcctgcgaggtgacccaccagggcctgagcagccccgtgaccaagagcttcaacaggggcgagtgcggtggaggtggatcagaattcggtatcgagcctttcagcggttccccaggcggcggctccgaaggcggcggaggtattgaaccttttagcggtggaggtggctccgaaggcggtggcgcgcccggtagcactagtggtattataccttttagcgcggccgcactgggcaagaagctgctggaggccgccagggccggccaggacgacgaggttaggatcctgatggccaacggcgccgacgtgaacgccatcgacactattggcctgacccccctgcacctggccgcccacgacggccacctggagatcgtggaggtgctgctgaagaacggagcagatgttaatgctgctgacaactggggcatcacccccctgcacctggccgcccggcgcggacatcttgaaattgtcgaagtcttgcttaaacacggtgctgacgtcaatgcagacgacgtgcagggcaacacccccctgcacctgaccgcccaccacggtcacttggagatagttgaggtacttctcaagcaaggagcagatgttaacgctcaggacaagttcggcaagaccgccttcgacatcagcatcgacaacggcaacgaggacctggccgagatcctgcagtaataatctaga

SEQ ID NO: 70 - protein, 439 aa, Artificial Sequence
  Description of Artificial Sequence: Synthetic polypeptide
MDWTWRILFLVAAATGAHSQIVLSQSPAILSASPGEKVTMTCRASSSVSYIHWFQQKPGSSPKPWIYATSNLASGVPVRFSGSGSGTSYSLTISRVEAEDAATYYCQQWTSNPPTFGGGTKLEIKRTVAAPSVFIFPPSDEQLKSGTASVVCLLNNFYPREAKVQWKVDNALQSGNSQESVTEQDSKDSTYSLSSTLTLSKADYEKHKVYACEVTHQGLSSPVTKSFNRGECGGGGSEFGIEPFSGSPGGGSEGGGGIEPFSGGGGSEGGGAPGSTSGIIPFSAAALGKKLLEAARAGQDDEVRILMANGADVNAIDTIGLTPLHLAAHDGHLEIVEVLLKNGADVNAADNWGITPLHLAARRGHLEIVEVLLKHGADVNADDVQGNTPLHLTAHHGHLEIVEVLLKQGADVNAQDKFGKTAFDISIDNGNEDLAEILQ

SEQ ID NO: 71 - protein, 5 aa, Artificial Sequence
  Description of Artificial Sequence: Synthetic peptide
DDDDK